European Patent Application EP 4 748 395 A1, published May 27, 2026. Title: 基于脑内磷稳态促进剂的疗法. Applicant: 中国科学院脑科学与智能技术卓越创新中心. The sequence listing filed with the application follows.

SEQUENCE LISTING (156 sequences)

SEQ ID NO: 1 - DNA, 3752 bp, Homo sapiens
  source 1..3752: mol_type = other DNA
agcgtgttcctgcctgctgcttggctgcagttaattttagccggggttagttctatgagttgtaaaagtagaagttagcaagctgaaatgtgacttctcggcctaatgtggtaggatatctattttagacttcagattgtgtttgtgatcaggagagcagtcttctgaagaattgtggctcagttttcttggaaactacttgaggagacatcacagctttcccagatcgggaggaaaaatatggaatgtgttttaccgctgactgaacacaaccaaatgaactgtcctgacagtagtttgcaaaccagcagctagcagtttgtccagcctctaacattgtccagcactttccagagcaaactcactgtttacaagaactcttggccttacgaagtttataacctcaagctttgtttatttaaaatattcctgcaaaagaaaagtacccggcacccactttccaaaatggccatggatgagtatttgtggatggtcattttgggtttcatcatagctttcatcttggccttttctgttggtgcaaacgatgttgccaactcctttggtacagccgtgggctctggtgtggtgaccttgaggcaggcatgcattttagcttcaatatttgaaaccaccggctccgtgttactaggcgccaaagtaggagaaaccattcgcaaaggtatcattgacgtgaacctgtacaacgagacggtggagactctcatggctggggaagttagtgccatggttggttccgctgtgtggcagctgattgcttccttcctgaggcttccaatctcaggaacgcactgcattgtgggttctactataggattctcactggtcgcaatcggtaccaaaggtgtgcagtggatggagcttgtcaagattgttgcttcttggtttatatctccactgttgtctggtttcatgtctggcctgctgtttgtactcatcagaattttcatcttaaaaaaggaagaccctgttcccaatggcctccgggcactcccagtattctatgctgctaccatagcaatcaatgtcttttccatcatgtacacaggagcaccagtgctcggccttgttctccccatgtgggccatagccctcatttcctttggtgtcgccctcctgttcgctttttttgtgtggctcttcgtgtgtccgtggatgcggaggaaaataacaggcaaattacaaaaagaaggtgctttatcacgagtatctgacgaaagcctcagtaaggttcaggaagcagagtccccagtatttaaagagctaccaggtgccaaggctaatgatgacagcaccatcccgctcacgggagcagcaggggagacactggggacctcggaaggcacttctgcgggcagccaccctcgggctgcatacggaagagcactgtccatgacccatggctctgtgaaatcgcccatctccaacggcaccttcggcttcgacggccacaccaggagcgacggtcatgtgtaccacaccgtgcacaaagactcggggctctacaaagatctgctgcacaaaatccacatcgacaggggccccgaggagaagccagcccaggaaagcaactaccggctgctgcgccgaaacaacagttacacctgctacaccgcagccatttgtgggctgccagtgcacgccacctttcgagctgcggactcatcggccccagaggacagtgagaagctggtgggcgacaccgtgtcctactccaagaagaggctgcgctacgacagctactcgagctactgtaacgcggtggcagaggcggagatcgaggcggaggagggcggcgtggagatgaagctggcgtcggagctggccgaccctgaccagccgcgagaggaccctgcagaggaggagaaggaggagaaggacgcacccgaggttcacctcctgttccatttcctgcaggtcctcaccgcctgtttcgggtcctttgctcacggcggcaatgacgtgagtaatgccatcggtcccctggtagccttgtggctgatttacaaacaaggcggggtaacgcaagaagcagctacacccgtctggctgctgttttatggaggagttggaatctgcacaggcctctgggtctgggggagaagagtgatccagaccatggggaaggacctcactcccatcacgccgtccagcggcttcacgatcgagctggcctcagccttcacagtggtgatcgcctccaacatcgggcttccagtcagcaccacgcactgtaaggtgggctcggtggtggccgtgggctggatccgctcccgcaaggctgtggactggcgcctctttcggaacatcttcgtggcctggttcgtgaccgtccctgtggctgggctgttcagcgctgctgtcatggctcttctcatgtatgggatccttccatatgtgtgatttgtcttcttccagctgcaaacagctaaagggatggtctggtgttggcgtgtgggagacatgtgtgctcgtgccgcacatacacatcctggccgtgcacggctctctcatgaccagctctctgcctcccttccaggaggctccatcccacactgttcacccaggctgcggagactcaccttcccgagctaacttaactactgtacataataatatgtattaaactggtatcgtggtgatataatgtggtgcagttacttatatattaaatatctattgtatccatagaataggcagcattatttcaaacatattcaagttgggagtggagatcattgcctagaagtcaatattcaataaatcttgtacataactatttcgatggcaaatgttaagccttctaaaaggaaagtgtagattggaaaatgattttttttccaaatgatgtttttgccttctaatatactgtaaggtaatgagcttcagaacaggcaacctgaccctgcagaggtcgcgtgctgtgggatgacagcgggacgggagctcacaagtgctttcactgaagatttgttcatatactgtgtattgattgttgtgtaatatatcatcattgcttttgtaaatacgtaaaactgtaattttttaatggtgtgcttcccttatacttttttgatcagagaattttggaaagtaccaaagaagcaggggaatcattggccagtgttacgttttcacattgtctgtctcccaccctcactgatcacgcctgccccagagcagtgtgtggcggtgacaccgtcacccagcatgcgccacgccgtggctcccaccagcagtgccaccgccaccacaccccagatcccacccaccttgcagtggcctttccttgtcatcagagtagagaatgcacaggtgttggtgagggcgtgtggctgagcactacatgtcaagtccagagtcagtttctatcccaattctccctgcagcctgaagaacggatccttgtctccaatgtcagcacaaaggaggctttttctgtgctttgacattctagcacttcagggatgagagggagggagaatcctggatgctggatggagtatttctctgaggcccacacaaagctggacacccccaggctctactccatcccattggagtctcttctttttttgatagcgggagggaggaagtacgactaatgttggagcctgaaactatggaaatgctgctaaaatttttatattgacaaacattttcttggtacttcattgtcatttttcattaatcaaccatattaaatttataataaaaaatgcccctcagaa

SEQ ID NO: 2 - DNA, 135 bp, Homo sapiens
  source 1..135: mol_type = other DNA
gtagagatgacgacacaacagacagctgatgtatacgggtaatttggttagggagaagagggttagagaggaattctaccaccttctgctttcaacaggacatatcctcttgtaggaagagtcctgcagcaggag

SEQ ID NO: 3 - DNA, 76 bp, Homo sapiens
  source 1..76: mol_type = other DNA
gtcctaaaacacgttgggagaggaaagagctcttccttgaagtagaactccatgtgagaaattgcaatggactttg

SEQ ID NO: 4 - DNA, 6878 bp, synthetic construct
  source 1..6878: mol_type = other DNA; note; note (original language) = 事件crpE2的minigenes构建体
gaggagacatcacagctttcccagatcgggaggaaaaatatggaatgtgttttaccgctgactgaacacaaccaaatgaactgtcctgacagtagtttgcaaaccagcagctagcagtttgtccagcctctaacattgtccagcactttccagagcaaactcactgtttacaagaactcttggccttacgaagtttataacctcaagctttgtttatttaaaatattcctgcaaaagaaaagtacccggcacccactttccaaaatggccatggatgagtatttgtggatggtcattttgggtttcatcatagctttcatcttggccttttctgttggtgcaaacgatgttgccaactcctttggtacagccgtgggctctggtgtggtgaccttgaggcaggcatgcattttagcttcaatatttgaaaccaccggctccgtgttactaggcgccaaagtaggagaaaccattcgcaaaggtatcattgacgtgaacctgtacaacgagacggtggagactctcatggctggggaagttagtgccatggttggtgagtagcctcttctctataccgatgggacatccgcccactgacccgcttccctgcagtactttgcccatatccataaatgtgatttttgctttggcttttcaaaaactggttggatgtttcacatttactctcttatttttgctttctgcatattaatttatgatttttaaagtgtttaaatatcaggcaaccatttattttctgaacttttgagcaaacttggttgctaaaatagatttcagctaagtgaatacttttcagaaagtacagaaaaagacctttgtagaacagcgctttattattttagagttgtttgaaggttgtctaagtgaatgtgttttcaaggttgatgtatgaaatttccaggaaggttgatttagatttttttcttaaggtttttcatcaattaggaggcaatgttttgaaaacttggatgtcaaaaataatatttattagtctaacttttatattcacagtttaagttctaaagaagttaccaaataaatcttaagtgcgtgtgtttcaagaaattctggtctcttacattatttgtcatccttttgttggcttttgttttgattttctgattctacctctgggagctccatttggtatgtttgttttgttttccggccaaaaaataatgtgcgtgttgcctggtgatagcatgaccttttattgcagtttcaagttgtctacatgaagtgtggaggtgtgtgaactgtgtgaataagcagagtggctggttggacagagtgatgtccccatggcctaagcggacacagatctcggccccgtgggtcttcccatcactgccctcgctacgacagaaaagaaccttcccggcaggcgtgtgttaagtgcagctgacaggattctttttctgcttgcctctaggtagagatgacgacacaacagacagctgatgtatacgggtaatttggttagggagaagagggttagagaggaattctaccaccttctgctttcaacaggacatatcctcttgtaggaagagtcctgcagcaggaggtaagatgctggtgtactaagaatacagccacattcccccgagttctttattttgtcacttacattttttcttttctttttttttttttttttgagacagagtcttgctctgtggcccaggctggagtgcaatagtgtgatctccgctcactgccacctccacctcctgggttcaagctattctctcacctcaccctccggagtagctgagactaaaggcgtgtgccaccgcacctggctaatttttgtatttttagtagagacagggtttcaccatgttggccaggctagtcttgaactcctgacctcaagcaatccacccaccatcacctctcaaagtgctgggattacaggcgtgagccaccacacctggcctgtcacatttcttaaacacctggaatttagagattattgaccaagttcacaatggcccaatctcatgttgttcgaggcgtctgataagaagcagcctgttgtactaaggaattgcatattcaccaagcactgtaggccagtaacacacaccagggagctcctacttctcagcttgacgctttgtgttgtaaagatgtcaggttcaactttgggaggcccccgagatgggcagaccacttgatcccaggagtttgagaccagtctgggcaacatagggagaccctgtctgtacaaaaaaactaaaaaattagctgggcatggtggcacatgcctgtagtcctagctgcttgggaggctgaagtgggaggattgcttgagcccaggaggttgaggctgcagtgagttgtgattgtgccactgcactccagcatgggcgacatagccagaccctgtctcaaaaaaaaaaaaaaaaaaatcaggttcaagatcactttcattccaacaactatagtcattattgaattttacttaccttcatggaacatatgtatatctcagcatagtcagatataatggaaatttctcttagaaaaataaccgttctttgtaaaattcacctttttagttgtgatagatatctaagatttaattccatcaagtggaaattaagatttttctagtcaggaaaatctgactagatgtgttgaaagtatgggacaaatcaagaaaaacactgacaaaattaaatctttttttttttttttgagacggaatctcgctttgttgcccaggctggagtgcagtggtgtgatctcggctcactgcaacctctgcctcctgggttcaagcgattctcctgcctcagcctcctaagtagctgggattacaggcacccgacaccacacccagctaatttttgtatttttggtagagatggggtttcaccatgttagtcaggctggtctcaaactcctgacctcgtgatcctcccaccttggcctcccaaagtgctgggattacaggcgtgagccaccacacccggccacaaagttaagtcttaactgaagtttttccttttgatggataaactttagaggcatggttctgcttattaaagaaatttgttagggaagccacgctgaagacctccgtgtgacagaagggttcatgaacaaggcttcatctgctcactctttctgcagacgggatcatttctccgttccccacccctggcgtttggctctttactgaaagaatgaaggatacttacctcaactagaatttgggtttaccaaagcaatttggggttttgcttgaataacttgattttgtttgctttggtttttaaacttttttttttttggtatgtggttaaatgaatctcaaagcctattttgttgggaatttgtatgagttacctagattcataaaatcgggttctttgccctgggagctataaatttaagatggtggtgtaattaccattggccaaaaccacagctgattctgtccagatgcctgaattctccagtcttcctcttctaaatccaacagtccttttttcttctccctctttccctctgtccttaattctattctgtttgcttcttttgttttctctgttagtcacttctccccaagcccctgggcgtctgtgcttcctgacagagttgtgttagagttaaggtgattgggtagaaattattgctgccagtgaaacgtcctgaacaagtcatcttgtgggactagctcagccctaaagcagtagtctgtccattttgtaggaaaccaccaatggttccaaaaatctgagaattcaaaactctgcatctttttttgtggaaagacccacactagcacaaacgagccagctcctcgaaacccttaagaagcacacagcccccttccagctccctctgcccagccacactctgccaccccacccccgcccggcagcctccctggagcctgagcctttgctctgccgtttctttcatctgcacgggaatggcggcctctgagatgcccatctccccactttccctaggtcgtggcttgcactcttatcccatgcttcatctctttcctctgtcagatgccattatcttacattaaagtatgtctttttccctctgttcttcctgacactaacatgatcccatttgtcttcagacacccctgaggctaaggtgctatcacctactcccaggccctcttgcaggtatttcctggccccaccaggccctccctcagctgtcccctgtctcctcccctccctgctatcctctctcctccttcttccctctctcaggtggtcccattactccctacctttctttacaaactctcctcctccaggatgtattttgtaaagtcagccacagaaaatatagcagctttcaggaaggacaaatcttatggtctgaattcaattgggtgggttgatatcactgtctcacatcatgagattattttaattgtaagaatataggctggtagcggtggctcacacctgtaatccgagcactttgggaggccgaggcaggcggatcatgaggtcaggagattgagaccatcttggctgacgcggtgaaaccccgtctctactaaaaatacaaaaaattagccgggcgtggtagcgggcacctgtagtcccagctactcgggaggctgaggcaggagaatggcgtgaacccaggaggcagagcttgcagtgagccgagattgcgcctgggcaacagagcaagaccccgtctaaaaaaaaaaaaaagaatataaaccatatcatgtattttctaagctatgaatccgtgctatgaaacgtgctccaaaccctggctttctttttaaaaccactagtccccgaggagcccagggctcagatgtggaggcttaaggaggtgtccgcgggtaggcctggcgctgccatggagcctgatatgggtttggcagcacaaggctggccccttctcctcccaacgcacgccttaaggattgacacagggtcacagccagcctcagctcaaaggtcagcacgcctagcactcatggcagcaactgtgtgtgttgcttcatggactgggtcctgcacagccataaatgatcctcctgcaactcagatgcctttgaaggaaatgccaggggtcccctgaaaagtgctgctgctgccaggcaaccaggtttccagaattaacgtttgggattaataacgtgcccagcttatcagccaggccctttgttcccctacagttccatgggagcttttcaacaactgcttctgaaagtgatctctcccggttgatgcttttaatactcactacaaaatctgatctgcttatgaaaatatttgaagtgaactgtagcctagaaaaacatgaaacctagaaaagagttggtgaaattgaggtaaaaggacacaaagccaacactaatgagaacctcttaacaacaaggaatcagacacacaaataaaaagtccaacattctgggtaggatctgagagcagatgcccaaatttgggttaaatatcatagttatttctcataggagaggcaccatcaacaagcagtatgggctgggtgcagtggctcactgcatccagtgagcctgtcatcccagcactttgggaggccatggtgggaaaatggcttgagcccaggagttcaagaccagccagggcaacatagcaagacccccgtctctgcaaaaaaattttaataattagctgagtgtggcagctcatgcctgtaatcccagggctttgggaggctgaagcaggaggattgcttaaggccaggagttccaaaccagcctgggtaacatagcaaaatcctgtctctgcaaaaaaatttaaaaattaaccaggtgtggtggtgcacacttgtaatctcagctgcttgggaggctgagacaggaggatcatttgagtccaggagtttaaggctgcagtgagccatgattttgcagctgtactccagcctgggcaagagtgagacgctgtctctacaaaagaaaaaaagaaaagaaaagaaaaaagcaacatggtattatactctcttatatagataatatgacctagccaatatctggtccttttcattatgtgactgtaaggcagaactacaacaaaatcttttcccaatatattgcctttctagtctttctgtgttcattcgagactttaatctcttgcttggttttggccaaaattcaccccagaacaagttcatacacagcaccctcactgaaaactgacaagggcagtcagtgtgtagcaccaggagacttgcctttaaatgcataatctggccggacacaatgcctcacgcatgtaatcccagcactttgggaggccaaggcgggtagatcacttgaggttaggggttcgagaccagcctggctaacatagtgagaccccatctttactaaaaatacaaaaattagccagagggcttgcttgaacccaggaggcagaggttgcagtgagccaagatcaggccactgcactccagcctgggcaacagagcaggactagcttcaaaaaataaataaataaccatcatccctgtcccctctgtgttgaggaaggcagaagctttcctttaactgaagttaattgagtgatttttgtccaggctgtagcgctttgtaaagaaacaattcacagaaaattaaactctgggagatgttgttatggaaaacatttggatttcttcccttggtgtctgcacctctgtactctgtatctgatggttttttgtccttcaatctgtaggttccgctgtgtggcagctgattgcttccttcctgaggcttccaatctcaggaacgcactgcattgtgggttctactataggattctcactggtcgcaatcggtaccaaaggtgtgcagtggatggagcttgtcaagattg

SEQ ID NO: 5 - DNA, 11040 bp, synthetic construct
  source 1..11040: mol_type = other DNA; note; note (original language) = 事件crpE10的minigenes构建体
cggcttcacgatcgagctggcctcagccttcacagtggtgatcgcctccaacatcgggcttccagtcagcaccacgcactgtaaggtaggcccctgctagccgggagcccttccccaggccgctgggacaggtccagggccaccggagcgcatgcaagggaagctgtagggctctgtagatggttgtgcaaaatgcagctccaggttctccaggtctccgggaccttgtattcctccatctgttccctccaccgtcctcctctcggcaggacgacactatctctcgttcagacctggcttttccaaggcagaatgccagggctggcctgcctgggactggcctgctatcctcccactgtttccacagtggagtttgattggcatcctgtgtgcgctgggcatacctgtgggctcacttgggagcctgccacttggtccagccaatgaggggactgggggttgacagtgttagaaattaacacaaatcatctctggaattgtaggacacagttgtttctggttttgttccttatatgatgttcaaagtgactatattgccataaattccccacgaggggtaattgctgatactgaccactgcggagtgctctgaaacctgcagctggacaagagagggctcctggtcatggtgtggaaagttggagctgcagggaggagccctgaagaccagtgaagaggaaatgggttccgggagtttcagggagtgatccacaggtggccagggtggggaggaccagaacccaggtggggaggaccagagccccggtctcatcacccaactctgcccagtatctgcagatacttctaaaatagctcaggtgagcctctgtatacagacaaactcaccagtctcaacaaagcgaaagtcactttgagatttttcctaggttcattcatttgtattattcaagaaaaactaattggtgtttgctgcttgggagcagagctctcagcaccaggaggaatatatgagccctcaaaacagacacagccacccacgtttctatttactcacaattttaagattccagccagtatgtttaaaagacaacgccaagcaaaggcaagtggcttcatgcttcaaacacccaggtcaggtggccctcacaagagtatctggagtggcccagcagcgtgtttcaaagctggggctccacgcatgaagaatcagcctcagtggaaagagtttgttttttccttttttgctaccatatacagaaatacttcaatttccacaaagtttctgtatacaaatccccccacttactgatcatcaggagagtgctgggtaccgtgctcaacaccacacgcatggcacaccgttccctctccacagcaagcctgtgggggcggaactgtcactcccagtccacaggtgaggagactgggttccctcagagttgagccgcttcccacatgcacacagccacatgtgatagatccaggattcagatcttcacctcaggccacacaccttctcgttcaggtccccatcagcaccattgtggtgcccgaccatggccaaggtgcctggggcaagcactccactggtggtctccccaagaagcttccccagcttcatagatgaggaaactgaggcagaggaaagttaagtaacgtgcccgagattacacagccagggagcagcccagctgaggctcccacatggacggcatggccagcgtcctcctccccggctccgcctggcaagcatggggaaggaaggcaggaagaggtgcaggtgtgcccgccacccattcattgtgagtttcctaatgtgggttatttaaaacttaccagagaagcacatattcactgaaatatttcaaacaatacaagactataaggaatgaaaagtgacatcttctctggactccacatcacttccattcactgtggtgtgtggagcgtggaggagacgcgtgtcactaaatacattcttttccaaggacacgggcttatgacttttctataggcatcagttgtcttttggaatgcttttaaacagatgtaatgccatctttttaatgattaacctacactaaagcaagactgctgaaggcagactcttctacaccagttgaaatagcttttttttgttttgttttgttttgttttgttttgtttttgagatggagtctcactctcatccaggctggagtgcggtggcatggtcccagctcaccgcagcctctgcctcctgagttcaagcagttctcctgcctcagcctccgggtagctgagattacaggcatgcaccaccacacccagctaatttttgtatttttagtagagacatggcttcaccatgttggcaaggctggtctcgaactcctgacctcaggtgatctgcctgcctcagcctcccaaagtgctgggattacaggcgtgagccaccgtgcctggcctgaaagagcttttgaaaaaacagcacaggtttggttcttccaggttggtgctacttagctaactgtatgagcagtctaatccgtttgtatgtatactgtatacagtgttggaatggacagtactgattttgctaataacactaaactctagaatacagtttataggaatagatgaaaagtataaaatgcttatttaaaaagccaaactcttgaattatctatatgcatgatttccccaatactgtattgatatatatactataatgatgtgtgactaagagatttacatccagtttgtacaggaccttagtgaatagatgtatatgttatcattatcctaaaatacctgtacaaagtacatgataaggttttttttttgagatggagtctcgctctgtcacccaggctggagtgcagtggcgccatctccactcactgcaagctccgcctcctgggttcatgccattctcctgcctcagcttcctgagtagctgggactacaggtgcccaccaccagctacttttttatatttttagtagagacggggtttcaccgtgttagccaggatggtctcgatctcctgacctcgtgatccgcccgcctcagcctcccaaagtgctgggattacagacatgagccaccgtgcccagccagttttgtttcctttgagctggtgatgagtagtattaggatagcttcttggcacttaaagcaggtctccctgaatgggactgcagcagggtgccatctataaaattgacaagacaggtcacaacttggatttgagtaagtttgtccgatatcattgatcgtggacttctggacaaagcctagagctattccctgtgagcactaaggacagagtctcagctctcaggaacttgccgtgtagttggagagcagatggctctcatcagagtccaaataatagaagtgctgagaagagctcacagttgtcattaccccataacacttattctctcatatcacatatttcccctgcacacaacagtccccaaatggcaaacgtgggatgaactatgagagctgtgggatggcgtgaagaatggggccctctgtaagtgagactgtgaatctggaaacattgaaagggtattgatgtccacatagagtcatagttgaattgcatcagttttcaggataattatcctgtgtttgatttttaagtttcatgcttagagccatctaatagaaagtagggagaagttggggacttggcaggaaataagatggaaactattgtttaaaatgaggtttttaatgtatctaggtagatgttattgatttatgcttccttctaagtgtacatggctaagtgcatagatttgttttgttttgttttgtttgagacagagtcttgctttgtggcccaggctggagtgcagtggcttgatcttggctcactgcgacctccgcctcctgggttcaagcagttttcctgcctcagcctcctgagtagctgagattacaggcatgcaccaccatggttggctaatttttgtatttttagtagaaatggggtttctccatgttagccaggctggtcttgaactcctgacctcaagtggtctgcctgcctcggcctcccaaagtgctggaattacaggcatgagccagtgcgcccggcctaagtgcatagtttcaattttgtcgtagcctatttcaaaacatttatgaaaccatactatattatgtgatatatgaactgaaggtataacttgggaaaaaacaattaggaaagtcctgttatcacattttattccagaaggcatatataaggcagtctgtttgatgagttacaccctctgtatgtattctggttttatatattttgtatttcatatcagaggactcagtttatcagatattttcctggaataatacctttgagtagggtcaaaagccttaattggccaggtacggtggctcatgcctataatcctagctactcgggaggctgaggccggagaatcgcttgaacccgggaggcggaggttgtggtgagtggagattgcaccattgcacttcagcctgggcaacaagagcaaaactatccccccccgcaccccccaaaaaaagccttaattgaagacacagaaaccggttttgaaaataaaagaatcctcagatgttatgtttcagcaattcgttcatcattcttcccttctgtgacccttaatcacgtttggtctttagccctagcagataacacacagtgccactactgagcacagttgctcatgtgtgtgctctttaataggaatttggaagtcatattctgcagaatgttttaattccatactgggtggattgagattattcctgtttgtggatcacccacattgtcagtcctcactgatgacatagatgatgattcaaccaccatttcaatttggaacagcatacagggaacactactgatttcaaatgtaggattataatttctaatttaatttctaattcttgttctctggtcccccttcttctcaacaattttttgctataagtacctgatgatggccttaaactggaaacacactcgatttattaaaagggaagttagaacacagcaaaaaaataacattttacattcacggaagacatgatcagtagcaaagacatagtactctggatcttttatgaatcaaataacatgtaactaaatacataaaattgttaagaactcagaaattactgtcttagcgtatgataaatgaagtatagaaaaagtatgtgggaatatgaagaatttgaacgtttatttagaacagcataattaataaatatgtacaagtttttacgctactgatcatatgccttcctgtcaagcatcgtgaaacatttataaaaatcctaaaatcagaagaccatgataaaaatctctataaaattttaaaaacagacctgacatggtggctcacacctgtaatcccagcactttgggaggcagaggtaggaggatcgcttgagcccagaagtttgaaaccagcctggggcaacatagtgagaccctgtctctattttataaaagttaaaatttaaattaaaaaaaaaaaaagtttaaagataagttgtgctaaccatgatctctaattacaataaaattaaactagaaattaattatatattgaaataagaatgtatcccaatggagactttttaatgcttttttaaggtaacaattgaattaaggagtttagaaaaatacaaggatagctttcttggaaaataataaaaaccaaatgtgtgtgtctgtgggtggatacaaacagcaaaacctgtggcaaccaagttatgctaagatgaaaattcatatctttaaatggtttaattgatcaaagggaaaataaaataaccaagtattaaaattaggattttgtaaaaagtccaggacagtaagaattgaggaaacaggttgtaagaaatatagaagcaaaattaatttaaaacaaaataagaaggggagaggaaagtggctactaacaaaatgtcagatcacatcaaggaaaagagggaggggaaggaggaagacattgtaacaacagagaagagaactgtttccattattaaataagccacacagctatatgctaagaatttgaaaacccatgtgaattattttctgcaacaatatacgtgacaaagaaatattggcctaagaagtagaaaaaagtggaaaatctgacccagaacaataggatgaaattaagggagttctccaaaaataattgttcccacctaaaaaagcaaaaaggggctaggggtggggcgggtgaggatactgctgactagaggaattcattagaatcttttccatttaaacaaaaaaaaacccagctctcacacgatctcaactttcccacaatgtaggaagaaaaacaaaactaaaaaacctctcccatttgtgctatggcgtacactgaataaccctaataccaaacctaatttaaaatatcacaaacaatgaaatctgtttaccgatgaatattgattgtaaaaactttaagcaagatgctgaaaaatgacatcaacaatatttggctgggcatggtggctcgtgcctgtaatcccagcactttgggaggctgaggtgggcagatcatctgaggtcaggagttcgagaccagcctggccaacatggcaaaaccccgtctctactaaaaatataaaaattaggcaagtgtggtggtgggtgcctgtaatcccagctactagggaggctgaggcaggagaatcgcttgaacccaggaggtggaggttgcagtgagctgagattgtgccactgcactccagcctgggcgacagagcaagactctatctcaaaacaaaacaatactatacaagaacctttcagcaggaccaaattgatcaagattaccagaaagtgggctcccttcgtgacagggcaggactgcatcacccaccaccagcaggctgtgcagggcaaggtcctcgcaggggctcaagttgggtatataggcagcttcagtataatatgccttagcaatccacttaaaaaaaaaaagatctctgttgagatataagccaaaaagacatttgatgatattcagtatttctttttttttgagacggagtttcactcgttacccaggctggagtgccataatggcatgatctcagctcaccacaacctccacctcccgggttcaagcaattctcctgcctcagcctcccgagtagctgggattacaggtgtgcagcaccacacccagctaattttgtatttttagtagagacggggtttctccatgttggtcaggctggtctcgaactcctgacctcaggtgatctgcccgcctcggcctcccaaagtgctgggattacaggcatgagccaccgcacccggccgatattcagtatttctaaaacactactagagttcgtaagagtgaccaagtccaaggtaaaaatagaaaaatccagcacttgttcatcagcaatagccaattagaaaatgtaacgggagggaaaaaaactgccaccataattgcagcaaaaataaaagttatctcagaataatcctaataagcactgtgagtgtcatcaggcacatggtgtgttcttatagtcccagctactcaggaggctgaaggtacgaggacagcctgaacccaggagttcaagaccagtctaggcaacatagtaagaccccatctctaaacaactaaataaataattttttaaaaaagaaatgtgagtgatatatatggaagaggcacaaaactgctcagaggtataaaaagataatctgaatatgagacgtaatgtgctattggatgggaaaaccagatgttgtaatgaagtcacttctccctaaatacaacctgaacaggattttacttggaattttacaaaacgagactaaagaatacattttggtgaaataaattatcagcaatataaaatgatctaacaagaaaactgaaaggaggaactagccttacctgacgtataatgtcatataaggaaacaaaagtcaagagtaggtcctgggaggaggggctagaactgggtgttagtgttttatggggcagtttccccgtgggatgatgaaaaagttctggagacagattgtggtgatggtttgcaaaacaatgtgattgtacttaatgcctctaaatggtatgctgaaaaattactaaaactgtaagttttatgttatgtatatcttaccacaataatttttaaaagtagatacctggataagaacagagtagatagcaatggatggaacctgttctatatgagcatgtattttgaaaaagggaaaatttaaccagtaagtgtttgaaaggttgaatagctgactgtcagtctagaaaaacaaaattagaccactctcaaaatacatgaacataaatctgatggcttaaataatattttaaaaatattcttaaatttagagtaaaatggaattttattttagaaaaataaaatggaattaaatatttatcaaatattcaagccaaggataaatcacagaagaaaattatagcatattttattgcatgaagttagaaacttgaaagtgaaacaaagcaaaatactaccttaagaaaatgtgtattcgatatcacagagttaatattattcagtgaagactacacataaataaataaggaacacattagattttagtatgtaaatggacaaaatacatgaagagacaatttttttttttttttgagacggagttttactctgtcacccaggctggagtgcagtggtgccatctcggctcactgcaacctccacctccccagttcaagcgattctcctgcctcagccacccaagtagctgggactacaggtgtgcaccaccacgcctagctaattttttgtatttttagtagagatggggtttcaccctgttagccagcatggtcttgatctcctgaccttgtatccgcccgccttggcctcccaaagtgctgggattacaagcatgagccactgcacctggccgacaatttgtatatgtgaaagctagagagagtgaaattcagtaaatatattttttaaagttcagccttaattgtaattaaagatacgcaaattaaaacagcaacagtgcatctttttgtcggttaattagccaaaaaaagagcaacttacatgatatcatgtgctgatattcacagattatggatgacactacattaacagctatttataaaactatttgtcattatgtattaaggtcctaaaacacgttgggagaggaaagagctcttccttgaagtagaactccatgtgagaaattgcaatggactttggtaaatcaccattttattttatttattttttattttatttttttttgagactgagtctcattctgttgtccaggctggagtgcagtatcgcgatcttggctcactgcaacctccacctcccaggttcaagtgagtagctgggattccaggtatgcaccaccacacctggctaattttttttatttttagtagagacagggtttcaccatgttggtcaggctggtctcgaactcctgacctcaggtgatccacccgcctcggcctcctgaagtgctgagattacaggcgtgagccaccatgcccggcctggtaaatcaccattttatagccatcgtcataaacattggattgtgaaatctttagcagaaggggaaagtgaggtttgataagatgcaggatattttaatcatattaaaaagtctcttcacagattgtggcaaatgtcaaaaaatagtgaattgggtaaagagaaaacaggagttcttgcagcttttctctaagttttgaattatttcaagatacattttaaatgttccctgttaactacagtcgatttcagggaatttttttttttttttttttttttgagacagagtctctctctgtcgcccaggttggagtgcagtggcatgatctccgctcactgcaagctcaatgcaagctccgcctcccaggttcacgccattctcccgcctcagcctcccaagtagctgggactacaggcgcctgccaccacgcctggctaatttttggtattcttagtagagacggggtttcaccgtgttagccaggatggtctccatctcctgacctcgtgatccgcccacctcagcctcccaaagtgctgggattacaggcggaagccaccgcgcacggccgggaatattatttttaaagccaaaatccaacctgggcacagtggctcacgcctgtaatcccagcactttgggaggctgaggcgggccgatcacttgaggccaggagtttgagaccagcctgaccaacatggcgaaaccccatctctactaaaaaatatgaaaattagctggatgtggtggtgcttgcctgtaatcccacctactcaggaggctgagacaggagaatcgcttgaacctgggagacatagcttgcagtgagctgagattgcaccactgtactccagcactttgggaggccaaggagggagggtcacttgaggtgaggagttccacatcagcgtggccaacatggtgaaaccccgtctctactaaaaatatgaaaattagccaagggtgatggcatgcgcctgtaatctcagctgctcaggaggctgaggcaggagaattgcttgaacctgggagatggaggttgcagtaagctgagatcacaccactgcactccagcctgggtgaagagtgagactgtctcaaaacaactatataaaacaactatataaagagctatatgctgaagagaagaatccccaaacaattctacctaaaatctaagctattttaaaagctttaacaaatgtaggggactgggtaatgttgtactagagcttgtttctgagattagcccatgtacattggtagagtgtagcctttgtggctcacctgtttttactttgcaatgtctgctcccacaggtgggctcggtggtggccgtgggctggatccgctcccgcaaggctgtggactggcgcctctttcggaacatcttcgtggcctggttcgtgaccgtccctgtggctgggctgttcagcgctgctgtcatggctcttctcatgtatgggatccttccatatgtgtga

SEQ ID NO: 6 - DNA, 3887 bp, Homo sapiens
  source 1..3887: mol_type = other DNA
agcgtgttcctgcctgctgcttggctgcagttaattttagccggggttagttctatgagttgtaaaagtagaagttagcaagctgaaatgtgacttctcggcctaatgtggtaggatatctattttagacttcagattgtgtttgtgatcaggagagcagtcttctgaagaattgtggctcagttttcttggaaactacttgaggagacatcacagctttcccagatcgggaggaaaaatatggaatgtgttttaccgctgactgaacacaaccaaatgaactgtcctgacagtagtttgcaaaccagcagctagcagtttgtccagcctctaacattgtccagcactttccagagcaaactcactgtttacaagaactcttggccttacgaagtttataacctcaagctttgtttatttaaaatattcctgcaaaagaaaagtacccggcacccactttccaaaatggccatggatgagtatttgtggatggtcattttgggtttcatcatagctttcatcttggccttttctgttggtgcaaacgatgttgccaactcctttggtacagccgtgggctctggtgtggtgaccttgaggcaggcatgcattttagcttcaatatttgaaaccaccggctccgtgttactaggcgccaaagtaggagaaaccattcgcaaaggtatcattgacgtgaacctgtacaacgagacggtggagactctcatggctggggaagttagtgccatggttggtagagatgacgacacaacagacagctgatgtatacgggtaatttggttagggagaagagggttagagaggaattctaccaccttctgctttcaacaggacatatcctcttgtaggaagagtcctgcagcaggaggttccgctgtgtggcagctgattgcttccttcctgaggcttccaatctcaggaacgcactgcattgtgggttctactataggattctcactggtcgcaatcggtaccaaaggtgtgcagtggatggagcttgtcaagattgttgcttcttggtttatatctccactgttgtctggtttcatgtctggcctgctgtttgtactcatcagaattttcatcttaaaaaaggaagaccctgttcccaatggcctccgggcactcccagtattctatgctgctaccatagcaatcaatgtcttttccatcatgtacacaggagcaccagtgctcggccttgttctccccatgtgggccatagccctcatttcctttggtgtcgccctcctgttcgctttttttgtgtggctcttcgtgtgtccgtggatgcggaggaaaataacaggcaaattacaaaaagaaggtgctttatcacgagtatctgacgaaagcctcagtaaggttcaggaagcagagtccccagtatttaaagagctaccaggtgccaaggctaatgatgacagcaccatcccgctcacgggagcagcaggggagacactggggacctcggaaggcacttctgcgggcagccaccctcgggctgcatacggaagagcactgtccatgacccatggctctgtgaaatcgcccatctccaacggcaccttcggcttcgacggccacaccaggagcgacggtcatgtgtaccacaccgtgcacaaagactcggggctctacaaagatctgctgcacaaaatccacatcgacaggggccccgaggagaagccagcccaggaaagcaactaccggctgctgcgccgaaacaacagttacacctgctacaccgcagccatttgtgggctgccagtgcacgccacctttcgagctgcggactcatcggccccagaggacagtgagaagctggtgggcgacaccgtgtcctactccaagaagaggctgcgctacgacagctactcgagctactgtaacgcggtggcagaggcggagatcgaggcggaggagggcggcgtggagatgaagctggcgtcggagctggccgaccctgaccagccgcgagaggaccctgcagaggaggagaaggaggagaaggacgcacccgaggttcacctcctgttccatttcctgcaggtcctcaccgcctgtttcgggtcctttgctcacggcggcaatgacgtgagtaatgccatcggtcccctggtagccttgtggctgatttacaaacaaggcggggtaacgcaagaagcagctacacccgtctggctgctgttttatggaggagttggaatctgcacaggcctctgggtctgggggagaagagtgatccagaccatggggaaggacctcactcccatcacgccgtccagcggcttcacgatcgagctggcctcagccttcacagtggtgatcgcctccaacatcgggcttccagtcagcaccacgcactgtaaggtgggctcggtggtggccgtgggctggatccgctcccgcaaggctgtggactggcgcctctttcggaacatcttcgtggcctggttcgtgaccgtccctgtggctgggctgttcagcgctgctgtcatggctcttctcatgtatgggatccttccatatgtgtgatttgtcttcttccagctgcaaacagctaaagggatggtctggtgttggcgtgtgggagacatgtgtgctcgtgccgcacatacacatcctggccgtgcacggctctctcatgaccagctctctgcctcccttccaggaggctccatcccacactgttcacccaggctgcggagactcaccttcccgagctaacttaactactgtacataataatatgtattaaactggtatcgtggtgatataatgtggtgcagttacttatatattaaatatctattgtatccatagaataggcagcattatttcaaacatattcaagttgggagtggagatcattgcctagaagtcaatattcaataaatcttgtacataactatttcgatggcaaatgttaagccttctaaaaggaaagtgtagattggaaaatgattttttttccaaatgatgtttttgccttctaatatactgtaaggtaatgagcttcagaacaggcaacctgaccctgcagaggtcgcgtgctgtgggatgacagcgggacgggagctcacaagtgctttcactgaagatttgttcatatactgtgtattgattgttgtgtaatatatcatcattgcttttgtaaatacgtaaaactgtaattttttaatggtgtgcttcccttatacttttttgatcagagaattttggaaagtaccaaagaagcaggggaatcattggccagtgttacgttttcacattgtctgtctcccaccctcactgatcacgcctgccccagagcagtgtgtggcggtgacaccgtcacccagcatgcgccacgccgtggctcccaccagcagtgccaccgccaccacaccccagatcccacccaccttgcagtggcctttccttgtcatcagagtagagaatgcacaggtgttggtgagggcgtgtggctgagcactacatgtcaagtccagagtcagtttctatcccaattctccctgcagcctgaagaacggatccttgtctccaatgtcagcacaaaggaggctttttctgtgctttgacattctagcacttcagggatgagagggagggagaatcctggatgctggatggagtatttctctgaggcccacacaaagctggacacccccaggctctactccatcccattggagtctcttctttttttgatagcgggagggaggaagtacgactaatgttggagcctgaaactatggaaatgctgctaaaatttttatattgacaaacattttcttggtacttcattgtcatttttcattaatcaaccatattaaatttataataaaaaatgcccctcagaa

SEQ ID NO: 7 - DNA, 3828 bp, Homo sapiens
  source 1..3828: mol_type = other DNA
agcgtgttcctgcctgctgcttggctgcagttaattttagccggggttagttctatgagttgtaaaagtagaagttagcaagctgaaatgtgacttctcggcctaatgtggtaggatatctattttagacttcagattgtgtttgtgatcaggagagcagtcttctgaagaattgtggctcagttttcttggaaactacttgaggagacatcacagctttcccagatcgggaggaaaaatatggaatgtgttttaccgctgactgaacacaaccaaatgaactgtcctgacagtagtttgcaaaccagcagctagcagtttgtccagcctctaacattgtccagcactttccagagcaaactcactgtttacaagaactcttggccttacgaagtttataacctcaagctttgtttatttaaaatattcctgcaaaagaaaagtacccggcacccactttccaaaatggccatggatgagtatttgtggatggtcattttgggtttcatcatagctttcatcttggccttttctgttggtgcaaacgatgttgccaactcctttggtacagccgtgggctctggtgtggtgaccttgaggcaggcatgcattttagcttcaatatttgaaaccaccggctccgtgttactaggcgccaaagtaggagaaaccattcgcaaaggtatcattgacgtgaacctgtacaacgagacggtggagactctcatggctggggaagttagtgccatggttggttccgctgtgtggcagctgattgcttccttcctgaggcttccaatctcaggaacgcactgcattgtgggttctactataggattctcactggtcgcaatcggtaccaaaggtgtgcagtggatggagcttgtcaagattgttgcttcttggtttatatctccactgttgtctggtttcatgtctggcctgctgtttgtactcatcagaattttcatcttaaaaaaggaagaccctgttcccaatggcctccgggcactcccagtattctatgctgctaccatagcaatcaatgtcttttccatcatgtacacaggagcaccagtgctcggccttgttctccccatgtgggccatagccctcatttcctttggtgtcgccctcctgttcgctttttttgtgtggctcttcgtgtgtccgtggatgcggaggaaaataacaggcaaattacaaaaagaaggtgctttatcacgagtatctgacgaaagcctcagtaaggttcaggaagcagagtccccagtatttaaagagctaccaggtgccaaggctaatgatgacagcaccatcccgctcacgggagcagcaggggagacactggggacctcggaaggcacttctgcgggcagccaccctcgggctgcatacggaagagcactgtccatgacccatggctctgtgaaatcgcccatctccaacggcaccttcggcttcgacggccacaccaggagcgacggtcatgtgtaccacaccgtgcacaaagactcggggctctacaaagatctgctgcacaaaatccacatcgacaggggccccgaggagaagccagcccaggaaagcaactaccggctgctgcgccgaaacaacagttacacctgctacaccgcagccatttgtgggctgccagtgcacgccacctttcgagctgcggactcatcggccccagaggacagtgagaagctggtgggcgacaccgtgtcctactccaagaagaggctgcgctacgacagctactcgagctactgtaacgcggtggcagaggcggagatcgaggcggaggagggcggcgtggagatgaagctggcgtcggagctggccgaccctgaccagccgcgagaggaccctgcagaggaggagaaggaggagaaggacgcacccgaggttcacctcctgttccatttcctgcaggtcctcaccgcctgtttcgggtcctttgctcacggcggcaatgacgtgagtaatgccatcggtcccctggtagccttgtggctgatttacaaacaaggcggggtaacgcaagaagcagctacacccgtctggctgctgttttatggaggagttggaatctgcacaggcctctgggtctgggggagaagagtgatccagaccatggggaaggacctcactcccatcacgccgtccagcggcttcacgatcgagctggcctcagccttcacagtggtgatcgcctccaacatcgggcttccagtcagcaccacgcactgtaaggtcctaaaacacgttgggagaggaaagagctcttccttgaagtagaactccatgtgagaaattgcaatggactttggtgggctcggtggtggccgtgggctggatccgctcccgcaaggctgtggactggcgcctctttcggaacatcttcgtggcctggttcgtgaccgtccctgtggctgggctgttcagcgctgctgtcatggctcttctcatgtatgggatccttccatatgtgtgatttgtcttcttccagctgcaaacagctaaagggatggtctggtgttggcgtgtgggagacatgtgtgctcgtgccgcacatacacatcctggccgtgcacggctctctcatgaccagctctctgcctcccttccaggaggctccatcccacactgttcacccaggctgcggagactcaccttcccgagctaacttaactactgtacataataatatgtattaaactggtatcgtggtgatataatgtggtgcagttacttatatattaaatatctattgtatccatagaataggcagcattatttcaaacatattcaagttgggagtggagatcattgcctagaagtcaatattcaataaatcttgtacataactatttcgatggcaaatgttaagccttctaaaaggaaagtgtagattggaaaatgattttttttccaaatgatgtttttgccttctaatatactgtaaggtaatgagcttcagaacaggcaacctgaccctgcagaggtcgcgtgctgtgggatgacagcgggacgggagctcacaagtgctttcactgaagatttgttcatatactgtgtattgattgttgtgtaatatatcatcattgcttttgtaaatacgtaaaactgtaattttttaatggtgtgcttcccttatacttttttgatcagagaattttggaaagtaccaaagaagcaggggaatcattggccagtgttacgttttcacattgtctgtctcccaccctcactgatcacgcctgccccagagcagtgtgtggcggtgacaccgtcacccagcatgcgccacgccgtggctcccaccagcagtgccaccgccaccacaccccagatcccacccaccttgcagtggcctttccttgtcatcagagtagagaatgcacaggtgttggtgagggcgtgtggctgagcactacatgtcaagtccagagtcagtttctatcccaattctccctgcagcctgaagaacggatccttgtctccaatgtcagcacaaaggaggctttttctgtgctttgacattctagcacttcagggatgagagggagggagaatcctggatgctggatggagtatttctctgaggcccacacaaagctggacacccccaggctctactccatcccattggagtctcttctttttttgatagcgggagggaggaagtacgactaatgttggagcctgaaactatggaaatgctgctaaaatttttatattgacaaacattttcttggtacttcattgtcatttttcattaatcaaccatattaaatttataataaaaaatgcccctcagaa

SEQ ID NO: 8 - DNA, 335 bp, Homo sapiens
  source 1..335: mol_type = other DNA
tgggtcttcccatcactgccctcgctacgacagaaaagaaccttcccggcaggcgtgtgttaagtgcagctgacaggattctttttctgcttgcctctaggtagagatgacgacacaacagacagctgatgtatacgggtaatttggttagggagaagagggttagagaggaattctaccaccttctgctttcaacaggacatatcctcttgtaggaagagtcctgcagcaggaggtaagatgctggtgtactaagaatacagccacattcccccgagttctttattttgtcacttacattttttcttttctttttttttttttttttgagacag

SEQ ID NO: 9 - DNA, 276 bp, Homo sapiens
  source 1..276: mol_type = other DNA
aaaagagcaacttacatgatatcatgtgctgatattcacagattatggatgacactacattaacagctatttataaaactatttgtcattatgtattaaggtcctaaaacacgttgggagaggaaagagctcttccttgaagtagaactccatgtgagaaattgcaatggactttggtaaatcaccattttattttatttattttttattttatttttttttgagactgagtctcattctgttgtccaggctggagtgcagtatcgcgatcttggc

SEQ ID NO: 10 - DNA, 6484 bp, synthetic construct
  source 1..6484: mol_type = other DNA; note; note (original language) = 人源化小鼠模型供体序列crpE2
tcctttggtacagccgtgggctctggtgtggtgaccttgaggcaggcatgcattttagcttcaatatttgaaaccaccggctccgtgttactaggcgccaaagtaggagaaaccattcgcaaaggtatcattgacgtgaacctgtacaacgagacggtggagactctcatggctggggaagttagtgccatggttggtgagtagcctcttctctataccgatgggacatccgcccactgacccgcttccctgcagtactttgcccatatccataaatgtgatttttgctttggcttttcaaaaactggttggatgtttcacatttactctcttatttttgctttctgcatattaatttatgatttttaaagtgtttaaatatcaggcaaccatttattttctgaacttttgagcaaacttggttgctaaaatagatttcagctaagtgaatacttttcagaaagtacagaaaaagacctttgtagaacagcgctttattattttagagttgtttgaaggttgtctaagtgaatgtgttttcaaggttgatgtatgaaatttccaggaaggttgatttagatttttttcttaaggtttttcatcaattaggaggcaatgttttgaaaacttggatgtcaaaaataatatttattagtctaacttttatattcacagtttaagttctaaagaagttaccaaataaatcttaagtgcgtgtgtttcaagaaattctggtctcttacattatttgtcatccttttgttggcttttgttttgattttctgattctacctctgggagctccatttggtatgtttgttttgttttccggccaaaaaataatgtgcgtgttgcctggtgatagcatgaccttttattgcagtttcaagttgtctacatgaagtgtggaggtgtgtgaactgtgtgaataagcagagtggctggttggacagagtgatgtccccatggcctaagcggacacagatctcggccccgtgggtcttcccatcactgccctcgctacgacagaaaagaaccttcccggcaggcgtgtgttaagtgcagctgacaggattctttttctgcttgcctctaggtagagatgacgacacaacagacagctgatgtatacgggtaatttggttagggagaagagggttagagaggaattctaccaccttctgctttcaacaggacatatcgtcttgtaggaagagtcctgcagcaggaggtaagatgctggtgtactaagaatacagccacattcccccgagttctttattttgtcacttacattttttcttttctttttttttttttttttgagacagagtcttgctctgtggcccaggctggagtgcaatagtgtgatctccgctcactgccacctccacctcctgggttcaagctattctctcacctcaccctccggagtagctgagactaaaggcgtgtgccaccgcacctggctaatttttgtatttttagtagagacagggtttcaccatgttggccaggctagtcttgaactcctgacctcaagcaatccacccaccatcacctctcaaagtgctgggattacaggcgtgagccaccacacctggcctgtcacatttcttaaacacctggaatttagagattattgaccaagttcacaatggcccaatctcatgttgttcgaggcgtctgataagaagcagcctgttgtactaaggaattgcatattcaccaagcactgtaggccagtaacacacaccagggagctcctacttctcagcttgacgctttgtgttgtaaagatgtcaggttcaactttgggaggcccccgagatgggcagaccacttgatcccaggagtttgagaccagtctgggcaacatagggagaccctgtctgtacaaaaaaactaaaaaattagctgggcatggtggcacatgcctgtagtcctagctgcttgggaggctgaagtgggaggattgcttgagcccaggaggttgaggctgcagtgagttgtgattgtgccactgcactccagcatgggcgacatagccagaccctgtctcaaaaaaaaaaaaaaaaaaatcaggttcaagatcactttcattccaacaactatagtcattattgaattttacttaccttcatggaacatatgtatatctcagcatagtcagatataatggaaatttctcttagaaaaataaccgttctttgtaaaattcacctttttagttgtgatagatatctaagatttaattccatcaagtggaaattaagatttttctagtcaggaaaatctgactagatgtgttgaaagtatgggacaaatcaagaaaaacactgacaaaattaaatctttttttttttttttgagacggaatctcgctttgttgcccaggctggagtgcagtggtgtgatctcggctcactgcaacctctgcctcctgggttcaagcgattctcctgcctcagcctcctaagtagctgggattacaggcacccgacaccacacccagctaatttttgtatttttggtagagatggggtttcaccatgttagtcaggctggtctcaaactcctgacctcgtgatcctcccaccttggcctcccaaagtgctgggattacaggcgtgagccaccacacccggccacaaagttaagtcttaactgaagtttttccttttgatggataaactttagaggcatggttctgcttattaaagaaatttgttagggaagccacgctgaagacctccgtgtgacagaagggttcatgaacaaggcttcatctgctcactctttctgcagacgggatcatttctccgttccccacccctggcgtttggctctttactgaaagaatgaaggatacttacctcaactagaatttgggtttaccaaagcaatttggggttttgcttgaataacttgattttgtttgctttggtttttaaacttttttttttttggtatgtggttaaatgaatctcaaagcctattttgttgggaatttgtatgagttacctagattcataaaatcgggttctttgccctgggagctataaatttaagatggtggtgtaattaccattggccaaaaccacagctgattctgtccagatgcctgaattctccagtcttcctcttctaaatccaacagtccttttttcttctccctctttccctctgtccttaattctattctgtttgcttcttttgttttctctgttagtcacttctccccaagcccctgggcgtctgtgcttcctgacagagttgtgttagagttaaggtgattgggtagaaattattgctgccagtgaaacgtcctgaacaagtcatcttgtgggactagctcagccctaaagcagtagtctgtccattttgtaggaaaccaccaatggttccaaaaatctgagaattcaaaactctgcatctttttttgtggaaagacccacactagcacaaacgagccagctcctcgaaacccttaagaagcacacagcccccttccagctccctctgcccagccacactctgccaccccacccccgcccggcagcctccctggagcctgagcctttgctctgccgtttctttcatctgcacgggaatggcggcctctgagatgcccatctccccactttccctaggtcgtggcttgcactcttatcccatgcttcatctctttcctctgtcagatgccattatcttacattaaagtatgtctttttccctctgttcttcctgacactaacatgatcccatttgtcttcagacacccctgaggctaaggtgctatcacctactcccaggccctcttgcaggtatttcctggccccaccaggccctccctcagctgtcccctgtctcctcccctccctgctatcctctctcctccttcttccctctctcaggtggtcccattactccctacctttctttacaaactctcctcctccaggatgtattttgtaaagtcagccacagaaaatatagcagctttcaggaaggacaaatcttatggtctgaattcaattgggtgggttgatatcactgtctcacatcatgagattattttaattgtaagaatataggctggtagcggtggctcacacctgtaatccgagcactttgggaggccgaggcaggcggatcatgaggtcaggagattgagaccatcttggctgacgcggtgaaaccccgtctctactaaaaatacaaaaaattagccgggcgtggtagcgggcacctgtagtcccagctactcgggaggctgaggcaggagaatggcgtgaacccaggaggcagagcttgcagtgagccgagattgcgcctgggcaacagagcaagaccccgtctaaaaaaaaaaaaaagaatataaaccatatcatgtattttctaagctatgaatccgtgctatgaaacgtgctccaaaccctggctttctttttaaaaccactagtccccgaggagcccagggctcagatgtggaggcttaaggaggtgtccgcgggtaggcctggcgctgccatggagcctgatatgggtttggcagcacaaggctggccccttctcctcccaacgcacgccttaaggattgacacagggtcacagccagcctcagctcaaaggtcagcacgcctagcactcatggcagcaactgtgtgtgttgcttcatggactgggtcctgcacagccataaatgatcctcctgcaactcagatgcctttgaaggaaatgccaggggtcccctgaaaagtgctgctgctgccaggcaaccaggtttccagaattaacgtttgggattaataacgtgcccagcttatcagccaggccctttgttcccctacagttccatgggagcttttcaacaactgcttctgaaagtgatctctcccggttgatgcttttaatactcactacaaaatctgatctgcttatgaaaatatttgaagtgaactgtagcctagaaaaacatgaaacctagaaaagagttggtgaaattgaggtaaaaggacacaaagccaacactaatgagaacctcttaacaacaaggaatcagacacacaaataaaaagtccaacattctgggtaggatctgagagcagatgcccaaatttgggttaaatatcatagttatttctcataggagaggcaccatcaacaagcagtatgggctgggtgcagtggctcactgcatccagtgagcctgtcatcccagcactttgggaggccatggtgggaaaatggcttgagcccaggagttcaagaccagccagggcaacatagcaagacccccgtctctgcaaaaaaattttaataattagctgagtgtggcagctcatgcctgtaatcccagggctttgggaggctgaagcaggaggattgcttaaggccaggagttccaaaccagcctgggtaacatagcaaaatcctgtctctgcaaaaaaatttaaaaattaaccaggtgtggtggtgcacacttgtaatctcagctgcttgggaggctgagacaggaggatcatttgagtccaggagtttaaggctgcagtgagccatgattttgcagctgtactccagcctgggcaagagtgagacgctgtctctacaaaagaaaaaaagaaaagaaaagaaaaaagcaacatggtattatactctcttatatagataatatgacctagccaatatctggtccttttcattatgtgactgtaaggcagaactacaacaaaatcttttcccaatatattgcctttctagtctttctgtgttcattcgagactttaatctcttgcttggttttggccaaaattcaccccagaacaagttcatacacagcaccctcactgaaaactgacaagggcagtcagtgtgtagcaccaggagacttgcctttaaatgcataatctggccggacacaatgcctcacgcatgtaatcccagcactttgggaggccaaggcgggtagatcacttgaggttaggggttcgagaccagcctggctaacatagtgagaccccatctttactaaaaatacaaaaattagccagagggcttgcttgaacccaggaggcagaggttgcagtgagccaagatcaggccactgcactccagcctgggcaacagagcaggactagcttcaaaaaataaataaataaccatcatccctgtcccctctgtgttgaggaaggcagaagctttcctttaactgaagttaattgagtgatttttgtccaggctgtagcgctttgtaaagaaacaattcacagaaaattaaactctgggagatgttgttatggaaaacatttggatttcttcccttggtgtctgcacctctgtactctgtatctgatggttttttgtccttcaatctgtaggttccgctgtgtggcagctgattgcttccttcctgaggcttccaatctcaggaacgcactgcattgtgggttctactataggattctcactggtcgcaatcggt

SEQ ID NO: 11 - DNA, 10892 bp, synthetic construct
  source 1..10892: mol_type = other DNA; note; note (original language) = 人源化小鼠模型供体序列crpE10
gcctccaacatcgggcttccagtcagcaccacgcactgtaaggtaggcccctgctagccgggagcccttccccaggccgctgggacaggtccagggccaccggagcgcatgcaagggaagctgtagggctctgtagatggttgtgcaaaatgcagctccaggttctccaggtctccgggaccttgtattcctccatctgttccctccaccgtcctcctctcggcaggacgacactatctctcgttcagacctggcttttccaaggcagaatgccagggctggcctgcctgggactggcctgctatcctcccactgtttccacagtggagtttgattggcatcctgtgtgcgctgggcatacctgtgggctcacttgggagcctgccacttggtccagccaatgaggggactgggggttgacagtgttagaaattaacacaaatcatctctggaattgtaggacacagttgtttctggttttgttccttatatgatgttcaaagtgactatattgccataaattccccacgaggggtaattgctgatactgaccactgcggagtgctctgaaacctgcagctggacaagagagggctcctggtcatggtgtggaaagttggagctgcagggaggagccctgaagaccagtgaagaggaaatgggttccgggagtttcagggagtgatccacaggtggccagggtggggaggaccagaacccaggtggggaggaccagagccccggtctcatcacccaactctgcccagtatctgcagatacttctaaaatagctcaggtgagcctctgtatacagacaaactcaccagtctcaacaaagcgaaagtcactttgagatttttcctaggttcattcatttgtattattcaagaaaaactaattggtgtttgctgcttgggagcagagctctcagcaccaggaggaatatatgagccctcaaaacagacacagccacccacgtttctatttactcacaattttaagattccagccagtatgtttaaaagacaacgccaagcaaaggcaagtggcttcatgcttcaaacacccaggtcaggtggccctcacaagagtatctggagtggcccagcagcgtgtttcaaagctggggctccacgcatgaagaatcagcctcagtggaaagagtttgttttttccttttttgctaccatatacagaaatacttcaatttccacaaagtttctgtatacaaatccccccacttactgatcatcaggagagtgctgggtaccgtgctcaacaccacacgcatggcacaccgttccctctccacagcaagcctgtgggggcggaactgtcactcccagtccacaggtgaggagactgggttccctcagagttgagccgcttcccacatgcacacagccacatgtgatagatccaggattcagatcttcacctcaggccacacaccttctcgttcaggtccccatcagcaccattgtggtgcccgaccatggccaaggtgcctggggcaagcactccactggtggtctccccaagaagcttccccagcttcatagatgaggaaactgaggcagaggaaagttaagtaacgtgcccgagattacacagccagggagcagcccagctgaggctcccacatggacggcatggccagcgtcctcctccccggctccgcctggcaagcatggggaaggaaggcaggaagaggtgcaggtgtgcccgccacccattcattgtgagtttcctaatgtgggttatttaaaacttaccagagaagcacatattcactgaaatatttcaaacaatacaagactataaggaatgaaaagtgacatcttctctggactccacatcacttccattcactgtggtgtgtggagcgtggaggagacgcgtgtcactaaatacattcttttccaaggacacgggcttatgacttttctataggcatcagttgtcttttggaatgcttttaaacagatgtaatgccatctttttaatgattaacctacactaaagcaagactgctgaaggcagactcttctacaccagttgaaatagcttttttttgttttgttttgttttgttttgttttgtttttgagatggagtctcactctcatccaggctggagtgcggtggcatggtcccagctcaccgcagcctctgcctcctgagttcaagcagttctcctgcctcagcctccgggtagctgagattacaggcatgcaccaccacacccagctaatttttgtatttttagtagagacatggcttcaccatgttggcaaggctggtctcgaactcctgacctcaggtgatctgcctgcctcagcctcccaaagtgctgggattacaggcgtgagccaccgtgcctggcctgaaagagcttttgaaaaaacagcacaggtttggttcttccaggttggtgctacttagctaactgtatgagcagtctaatccgtttgtatgtatactgtatacagtgttggaatggacagtactgattttgctaataacactaaactctagaatacagtttataggaatagatgaaaagtataaaatgcttatttaaaaagccaaactcttgaattatctatatgcatgatttccccaatactgtattgatatatatactataatgatgtgtgactaagagatttacatccagtttgtacaggaccttagtgaatagatgtatatgttatcattatcctaaaatacctgtacaaagtacatgataaggttttttttttgagatggagtctcgctctgtcacccaggctggagtgcagtggcgccatctccactcactgcaagctccgcctcctgggttcatgccattctcctgcctcagcttcctgagtagctgggactacaggtgcccaccaccagctacttttttatatttttagtagagacggggtttcaccgtgttagccaggatggtctcgatctcctgacctcgtgatccgcccgcctcagcctcccaaagtgctgggattacagacatgagccaccgtgcccagccagttttgtttcctttgagctggtgatgagtagtattaggatagcttcttggcacttaaagcaggtctccctgaatgggactgcagcagggtgccatctataaaattgacaagacaggtcacaacttggatttgagtaagtttgtccgatatcattgatcgtggacttctggacaaagcctagagctattccctgtgagcactaaggacagagtctcagctctcaggaacttgccgtgtagttggagagcagatggctctcatcagagtccaaataatagaagtgctgagaagagctcacagttgtcattaccccataacacttattctctcatatcacatatttcccctgcacacaacagtccccaaatggcaaacgtgggatgaactatgagagctgtgggatggcgtgaagaatggggccctctgtaagtgagactgtgaatctggaaacattgaaagggtattgatgtccacatagagtcatagttgaattgcatcagttttcaggataattatcctgtgtttgatttttaagtttcatgcttagagccatctaatagaaagtagggagaagttggggacttggcaggaaataagatggaaactattgtttaaaatgaggtttttaatgtatctaggtagatgttattgatttatgcttccttctaagtgtacatggctaagtgcatagatttgttttgttttgttttgtttgagacagagtcttgctttgtggcccaggctggagtgcagtggcttgatcttggctcactgcgacctccgcctcctgggttcaagcagttttcctgcctcagcctcctgagtagctgagattacaggcatgcaccaccatggttggctaatttttgtatttttagtagaaatggggtttctccatgttagccaggctggtcttgaactcctgacctcaagtggtctgcctgcctcggcctcccaaagtgctggaattacaggcatgagccagtgcgcccggcctaagtgcatagtttcaattttgtcgtagcctatttcaaaacatttatgaaaccatactatattatgtgatatatgaactgaaggtataacttgggaaaaaacaattaggaaagtcctgttatcacattttattccagaaggcatatataaggcagtctgtttgatgagttacaccctctgtatgtattctggttttatatattttgtatttcatatcagaggactcagtttatcagatattttcctggaataatacctttgagtagggtcaaaagccttaattggccaggtacggtggctcatgcctataatcctagctactcgggaggctgaggccggagaatcgcttgaacccgggaggcggaggttgtggtgagtggagattgcaccattgcacttcagcctgggcaacaagagcaaaactatccccccccgcaccccccaaaaaaagccttaattgaagacacagaaaccggttttgaaaataaaagaatcctcagatgttatgtttcagcaattcgttcatcattcttcccttctgtgacccttaatcacgtttggtctttagccctagcagataacacacagtgccactactgagcacagttgctcatgtgtgtgctctttaataggaatttggaagtcatattctgcagaatgttttaattccatactgggtggattgagattattcctgtttgtggatcacccacattgtcagtcctcactgatgacatagatgatgattcaaccaccatttcaatttggaacagcatacagggaacactactgatttcaaatgtaggattataatttctaatttaatttctaattcttgttctctggtcccccttcttctcaacaattttttgctataagtacctgatgatggccttaaactggaaacacactcgatttattaaaagggaagttagaacacagcaaaaaaataacattttacattcacggaagacatgatcagtagcaaagacatagtactctggatcttttatgaatcaaataacatgtaactaaatacataaaattgttaagaactcagaaattactgtcttagcgtatgataaatgaagtatagaaaaagtatgtgggaatatgaagaatttgaacgtttatttagaacagcataattaataaatatgtacaagtttttacgctactgatcatatgccttcctgtcaagcatcgtgaaacatttataaaaatcctaaaatcagaagaccatgataaaaatctctataaaattttaaaaacagacctgacatggtggctcacacctgtaatcccagcactttgggaggcagaggtaggaggatcgcttgagcccagaagtttgaaaccagcctggggcaacatagtgagaccctgtctctattttataaaagttaaaatttaaattaaaaaaaaaaaaagtttaaagataagttgtgctaaccatgatctctaattacaataaaattaaactagaaattaattatatattgaaataagaatgtatcccaatggagactttttaatgcttttttaaggtaacaattgaattaaggagtttagaaaaatacaaggatagctttcttggaaaataataaaaaccaaatgtgtgtgtctgtgggtggatacaaacagcaaaacctgtggcaaccaagttatgctaagatgaaaattcatatctttaaatggtttaattgatcaaagggaaaataaaataaccaagtattaaaattaggattttgtaaaaagtccaggacagtaagaattgaggaaacaggttgtaagaaatatagaagcaaaattaatttaaaacaaaataagaaggggagaggaaagtggctactaacaaaatgtcagatcacatcaaggaaaagagggaggggaaggaggaagacattgtaacaacagagaagagaactgtttccattattaaataagccacacagctatatgctaagaatttgaaaacccatgtgaattattttctgcaacaatatacgtgacaaagaaatattggcctaagaagtagaaaaaagtggaaaatctgacccagaacaataggatgaaattaagggagttctccaaaaataattgttcccacctaaaaaagcaaaaaggggctaggggtggggcgggtgaggatactgctgactagaggaattcattagaatcttttccatttaaacaaaaaaaaacccagctctcacacgatctcaactttcccacaatgtaggaagaaaaacaaaactaaaaaacctctcccatttgtgctatggcgtacactgaataaccctaataccaaacctaatttaaaatatcacaaacaatgaaatctgtttaccgatgaatattgattgtaaaaactttaagcaagatgctgaaaaatgacatcaacaatatttggctgggcatggtggctcgtgcctgtaatcccagcactttgggaggctgaggtgggcagatcatctgaggtcaggagttcgagaccagcctggccaacatggcaaaaccccgtctctactaaaaatataaaaattaggcaagtgtggtggtgggtgcctgtaatcccagctactagggaggctgaggcaggagaatcgcttgaacccaggaggtggaggttgcagtgagctgagattgtgccactgcactccagcctgggcgacagagcaagactctatctcaaaacaaaacaatactatacaagaacctttcagcaggaccaaattgatcaagattaccagaaagtgggctcccttcgtgacagggcaggactgcatcacccaccaccagcaggctgtgcagggcaaggtcctcgcaggggctcaagttgggtatataggcagcttcagtataatatgccttagcaatccacttaaaaaaaaaaagatctctgttgagatataagccaaaaagacatttgatgatattcagtatttctttttttttgagacggagtttcactcgttacccaggctggagtgccataatggcatgatctcagctcaccacaacctccacctcccgggttcaagcaattctcctgcctcagcctcccgagtagctgggattacaggtgtgcagcaccacacccagctaattttgtatttttagtagagacggggtttctccatgttggtcaggctggtctcgaactcctgacctcaggtgatctgcccgcctcggcctcccaaagtgctgggattacaggcatgagccaccgcacccggccgatattcagtatttctaaaacactactagagttcgtaagagtgaccaagtccaaggtaaaaatagaaaaatccagcacttgttcatcagcaatagccaattagaaaatgtaacgggagggaaaaaaactgccaccataattgcagcaaaaataaaagttatctcagaataatcctaataagcactgtgagtgtcatcaggcacatggtgtgttcttatagtcccagctactcaggaggctgaaggtacgaggacagcctgaacccaggagttcaagaccagtctaggcaacatagtaagaccccatctctaaacaactaaataaataattttttaaaaaagaaatgtgagtgatatatatggaagaggcacaaaactgctcagaggtataaaaagataatctgaatatgagacgtaatgtgctattggatgggaaaaccagatgttgtaatgaagtcacttctccctaaatacaacctgaacaggattttacttggaattttacaaaacgagactaaagaatacattttggtgaaataaattatcagcaatataaaatgatctaacaagaaaactgaaaggaggaactagccttacctgacgtataatgtcatataaggaaacaaaagtcaagagtaggtcctgggaggaggggctagaactgggtgttagtgttttatggggcagtttccccgtgggatgatgaaaaagttctggagacagattgtggtgatggtttgcaaaacaatgtgattgtacttaatgcctctaaatggtatgctgaaaaattactaaaactgtaagttttatgttatgtatatcttaccacaataatttttaaaagtagatacctggataagaacagagtagatagcaatggatggaacctgttctatatgagcatgtattttgaaaaagggaaaatttaaccagtaagtgtttgaaaggttgaatagctgactgtcagtctagaaaaacaaaattagaccactctcaaaatacatgaacataaatctgatggcttaaataatattttaaaaatattcttaaatttagagtaaaatggaattttattttagaaaaataaaatggaattaaatatttatcaaatattcaagccaaggataaatcacagaagaaaattatagcatattttattgcatgaagttagaaacttgaaagtgaaacaaagcaaaatactaccttaagaaaatgtgtattcgatatcacagagttaatattattcagtgaagactacacataaataaataaggaacacattagattttagtatgtaaatggacaaaatacatgaagagacaatttttttttttttttgagacggagttttactctgtcacccaggctggagtgcagtggtgccatctcggctcactgcaacctccacctccccagttcaagcgattctcctgcctcagccacccaagtagctgggactacaggtgtgcaccaccacgcctagctaattttttgtatttttagtagagatggggtttcaccctgttagccagcatggtcttgatctcctgaccttgtatccgcccgccttggcctcccaaagtgctgggattacaagcatgagccactgcacctggccgacaatttgtatatgtgaaagctagagagagtgaaattcagtaaatatattttttaaagttcagccttaattgtaattaaagatacgcaaattaaaacagcaacagtgcatctttttgtcggttaattagccaaaaaaagagcaacttacatgatatcatgtgctgatattcacagattatggatgacactacattaacagctatttataaaactatttgtcattatgtattaaggtcctaaaacacgttgggagaggaaagagctcttccttgaagtagaactccatgtgagaaattgcaatggactttggtaaatcaccattttattttatttattttttattttatttttttttgagactgagtctcattctgttgtccaggctggagtgcagtatcgcgatcttggctcactgcaacctccacctcccaggttcaagtgagtagctgggattccaggtatgcaccaccacacctggctaattttttttatttttagtagagacagggtttcaccatgttggtcaggctggtctcgaactcctgacctcaggtgatccacccgcctcggcctcctgaagtgctgagattacaggcgtgagccaccatgcccggcctggtaaatcaccattttatagccatcgtcataaacattggattgtgaaatctttagcagaaggggaaagtgaggtttgataagatgcaggatattttaatcatattaaaaagtctcttcacagattgtggcaaatgtcaaaaaatagtgaattgggtaaagagaaaacaggagttcttgcagcttttctctaagttttgaattatttcaagatacattttaaatgttccctgttaactacagtcgatttcagggaatttttttttttttttttttttttgagacagagtctctctctgtcgcccaggttggagtgcagtggcatgatctccgctcactgcaagctcaatgcaagctccgcctcccaggttcacgccattctcccgcctcagcctcccaagtagctgggactacaggcgcctgccaccacgcctggctaatttttggtattcttagtagagacggggtttcaccgtgttagccaggatggtctccatctcctgacctcgtgatccgcccacctcagcctcccaaagtgctgggattacaggcggaagccaccgcgcacggccgggaatattatttttaaagccaaaatccaacctgggcacagtggctcacgcctgtaatcccagcactttgggaggctgaggcgggccgatcacttgaggccaggagtttgagaccagcctgaccaacatggcgaaaccccatctctactaaaaaatatgaaaattagctggatgtggtggtgcttgcctgtaatcccacctactcaggaggctgagacaggagaatcgcttgaacctgggagacatagcttgcagtgagctgagattgcaccactgtactccagcactttgggaggccaaggagggagggtcacttgaggtgaggagttccacatcagcgtggccaacatggtgaaaccccgtctctactaaaaatatgaaaattagccaagggtgatggcatgcgcctgtaatctcagctgctcaggaggctgaggcaggagaattgcttgaacctgggagatggaggttgcagtaagctgagatcacaccactgcactccagcctgggtgaagagtgagactgtctcaaaacaactatataaaacaactatataaagagctatatgctgaagagaagaatccccaaacaattctacctaaaatctaagctattttaaaagctttaacaaatgtaggggactgggtaatgttgtactagagcttgtttctgagattagcccatgtacattggtagagtgtagcctttgtggctcacctgtttttactttgcaatgtctgctcccacaggtgggctcggtggtggccgtgggctggatccgctcccgcaaggctgtggactggcgcctc

SEQ ID NO: 12 - DNA, 20 bp, synthetic construct
  source 1..20: mol_type = other DNA; note = ASO
gtcatctctacctagaggca

SEQ ID NO: 13 - DNA, 20 bp, synthetic construct
  source 1..20: mol_type = other DNA; note = ASO
tagaggcaagcagaaaaaga

SEQ ID NO: 14 - DNA, 20 bp, synthetic construct
  source 1..20: mol_type = other DNA; note = ASO
tctacctagaggcaagcaga

SEQ ID NO: 15 - DNA, 20 bp, synthetic construct
  source 1..20: mol_type = other DNA; note = ASO
ctctacctagaggcaagcag

SEQ ID NO: 16 - DNA, 20 bp, synthetic construct
  source 1..20: mol_type = other DNA; note = ASO
tctctacctagaggcaagca

SEQ ID NO: 17 - DNA, 20 bp, synthetic construct
  source 1..20: mol_type = other DNA; note = ASO
atctctacctagaggcaagc

SEQ ID NO: 18 - DNA, 20 bp, synthetic construct
  source 1..20: mol_type = other DNA; note = ASO
catctctacctagaggcaag

SEQ ID NO: 19 - DNA, 20 bp, synthetic construct
  source 1..20: mol_type = other DNA; note = ASO
tcatctctacctagaggcaa

SEQ ID NO: 20 - DNA, 20 bp, synthetic construct
  source 1..20: mol_type = other DNA; note = ASO
gtcatctctacctagaggca

SEQ ID NO: 21 - DNA, 20 bp, synthetic construct
  source 1..20: mol_type = other DNA; note = ASO
cgtcatctctacctagaggc

SEQ ID NO: 22 - DNA, 20 bp, synthetic construct
  source 1..20: mol_type = other DNA; note = ASO
tcgtcatctctacctagagg

SEQ ID NO: 23 - DNA, 22 bp, synthetic construct
  source 1..22: mol_type = other DNA; note = ASO
tcgtcatctctacctagaggca

SEQ ID NO: 24 - DNA, 18 bp, synthetic construct
  source 1..18: mol_type = other DNA; note = ASO
tcgtcatctctacctaga

SEQ ID NO: 25 - DNA, 20 bp, synthetic construct
  source 1..20: mol_type = other DNA; note = ASO
gtcgtcatctctacctagag

SEQ ID NO: 26 - DNA, 20 bp, synthetic construct
  source 1..20: mol_type = other DNA; note = ASO
tgtcgtcatctctacctaga

SEQ ID NO: 27 - DNA, 20 bp, synthetic construct
  source 1..20: mol_type = other DNA; note = ASO
gtgtcgtcatctctacctag

SEQ ID NO: 28 - DNA, 20 bp, synthetic construct
  source 1..20: mol_type = other DNA; note = ASO
tgtgtcgtcatctctaccta

SEQ ID NO: 29 - DNA, 20 bp, synthetic construct
  source 1..20: mol_type = other DNA; note = ASO
ttgtgtcgtcatctctacct

SEQ ID NO: 30 - DNA, 20 bp, synthetic construct
  source 1..20: mol_type = other DNA; note = ASO
gttgtgtcgtcatctctacc

SEQ ID NO: 31 - DNA, 20 bp, synthetic construct
  source 1..20: mol_type = other DNA; note = ASO
tgttgtgtcgtcatctctac

SEQ ID NO: 32 - DNA, 20 bp, synthetic construct
  source 1..20: mol_type = other DNA; note = ASO
ctgttgtgtcgtcatctcta

SEQ ID NO: 33 - DNA, 21 bp, synthetic construct
  source 1..21: mol_type = other DNA; note = ASO
tctgttgtgtcgtcatctcta

SEQ ID NO: 34 - DNA, 20 bp, synthetic construct
  source 1..20: mol_type = other DNA; note = ASO
gtctgttgtgtcgtcatctc

SEQ ID NO: 35 - DNA, 20 bp, synthetic construct
  source 1..20: mol_type = other DNA; note = ASO
tgtctgttgtgtcgtcatct

SEQ ID NO: 36 - DNA, 21 bp, synthetic construct
  source 1..21: mol_type = other DNA; note = ASO
tacaccagcatcttacctcct

SEQ ID NO: 37 - DNA, 20 bp, synthetic construct
  source 1..20: mol_type = other DNA; note = ASO
ccagcatcttacctcctgct

SEQ ID NO: 38 - DNA, 20 bp, synthetic construct
  source 1..20: mol_type = other DNA; note = ASO
cagcatcttacctcctgctg

SEQ ID NO: 39 - DNA, 20 bp, synthetic construct
  source 1..20: mol_type = other DNA; note = ASO
agcatcttacctcctgctgc

SEQ ID NO: 40 - DNA, 20 bp, synthetic construct
  source 1..20: mol_type = other DNA; note = ASO
gcatcttacctcctgctgca

SEQ ID NO: 41 - DNA, 20 bp, synthetic construct
  source 1..20: mol_type = other DNA; note = ASO
catcttacctcctgctgcag

SEQ ID NO: 42 - DNA, 20 bp, synthetic construct
  source 1..20: mol_type = other DNA; note = ASO
atcttacctcctgctgcagg

SEQ ID NO: 43 - DNA, 20 bp, synthetic construct
  source 1..20: mol_type = other DNA; note = ASO
tcttacctcctgctgcagga

SEQ ID NO: 44 - DNA, 20 bp, synthetic construct
  source 1..20: mol_type = other DNA; note = ASO
cttacctcctgctgcaggac

SEQ ID NO: 45 - DNA, 20 bp, synthetic construct
  source 1..20: mol_type = other DNA; note = ASO
ttacctcctgctgcaggact

SEQ ID NO: 46 - DNA, 21 bp, synthetic construct
  source 1..21: mol_type = other DNA; note = ASO
taggaccttaatacataatga

SEQ ID NO: 47 - DNA, 20 bp, synthetic construct
  source 1..20: mol_type = other DNA; note = ASO
ttttaggaccttaatacata

SEQ ID NO: 48 - DNA, 20 bp, synthetic construct
  source 1..20: mol_type = other DNA; note = ASO
gttttaggaccttaatacat

SEQ ID NO: 49 - DNA, 20 bp, synthetic construct
  source 1..20: mol_type = other DNA; note = ASO
tgttttaggaccttaataca

SEQ ID NO: 50 - DNA, 20 bp, synthetic construct
  source 1..20: mol_type = other DNA; note = ASO
gtgttttaggaccttaatac

SEQ ID NO: 51 - DNA, 20 bp, synthetic construct
  source 1..20: mol_type = other DNA; note = ASO
cgtgttttaggaccttaata

SEQ ID NO: 52 - DNA, 20 bp, synthetic construct
  source 1..20: mol_type = other DNA; note = ASO
acgtgttttaggaccttaat

SEQ ID NO: 53 - DNA, 20 bp, synthetic construct
  source 1..20: mol_type = other DNA; note = ASO
aacgtgttttaggaccttaa

SEQ ID NO: 54 - DNA, 20 bp, synthetic construct
  source 1..20: mol_type = other DNA; note = ASO
caacgtgttttaggacctta

SEQ ID NO: 55 - DNA, 21 bp, synthetic construct
  source 1..21: mol_type = other DNA; note = ASO
tcccaacgtgttttaggacct

SEQ ID NO: 56 - DNA, 20 bp, synthetic construct
  source 1..20: mol_type = other DNA; note = ASO
tggtgatttaccaaagtcca

SEQ ID NO: 57 - DNA, 22 bp, synthetic construct
  source 1..22: mol_type = other DNA; note = ASO
tgatttaccaaagtccattgca

SEQ ID NO: 58 - DNA, 20 bp, synthetic construct
  source 1..20: mol_type = other DNA; note = ASO
tttaccaaagtccattgcaa

SEQ ID NO: 59 - DNA, 20 bp, synthetic construct
  source 1..20: mol_type = other DNA; note = ASO
acgtgtttcaggaccttaat

SEQ ID NO: 60 - DNA, 18 bp, synthetic construct
  source 1..18: mol_type = other DNA; note = ASO
gtgtttcaggaccttaat

SEQ ID NO: 61 - DNA, 20 bp, synthetic construct
  source 1..20: mol_type = other DNA; note = ASO
gtttcaggaccttaatacat

SEQ ID NO: 62 - DNA, 25 bp, synthetic construct
  source 1..25: mol_type = other DNA; note = ASO
cctcttacctcagttacaatttata

SEQ ID NO: 63 - DNA, 25 bp, synthetic construct
  source 1..25: mol_type = other DNA; note = ASO
tcatctctacctagaggcaagcaga

SEQ ID NO: 64 - DNA, 25 bp, synthetic construct
  source 1..25: mol_type = other DNA; note = ASO
catctctacctagaggcaagcagaa

SEQ ID NO: 65 - DNA, 25 bp, synthetic construct
  source 1..25: mol_type = other DNA; note = ASO
atctctacctagaggcaagcagaaa

SEQ ID NO: 66 - DNA, 25 bp, synthetic construct
  source 1..25: mol_type = other DNA; note = ASO
ttcaggaccttaatacataatgaca

SEQ ID NO: 67 - DNA, 25 bp, synthetic construct
  source 1..25: mol_type = other DNA; note = ASO
gtttcaggaccttaatacataatga

SEQ ID NO: 68 - DNA, 25 bp, synthetic construct
  source 1..25: mol_type = other DNA; note = ASO
tttcaggaccttaatacataatgac

SEQ ID NO: 69 - DNA, 41 bp, synthetic construct
  source 1..41: mol_type = other DNA; note = primer
tagggcggccgggaattggatcacaggaggagacatcacag

SEQ ID NO: 70 - DNA, 21 bp, synthetic construct
  source 1..21: mol_type = other DNA; note = primer
gatatgtcctgttgaaagcag

SEQ ID NO: 71 - DNA, 25 bp, synthetic construct
  source 1..25: mol_type = other DNA; note = primer
gctttcaacaggacatatcctcttg

SEQ ID NO: 72 - DNA, 20 bp, synthetic construct
  source 1..20: mol_type = other DNA; note = primer
cgacctagggaaagtgggga

SEQ ID NO: 73 - DNA, 20 bp, synthetic construct
  source 1..20: mol_type = other DNA; note = primer
ccccactttccctaggtcgt

SEQ ID NO: 74 - DNA, 45 bp, synthetic construct
  source 1..45: mating_type = primer; mol_type = other DNA
gcgatcgcagatccttgcggccttaccaatcttgacaagctccat

SEQ ID NO: 75 - DNA, 39 bp, synthetic construct
  source 1..39: mol_type = other DNA; note = primer
ctttcaacaggacatatcgtcttgtaggaagagtcctgc

SEQ ID NO: 76 - DNA, 40 bp, synthetic construct
  source 1..40: mol_type = other DNA; note = primer
caagacgatatgtcctgttgaaagcagaaggtggtagaat

SEQ ID NO: 77 - DNA, 38 bp, synthetic construct
  source 1..38: mol_type = other DNA; note = primer
gtatacaggtaatttggttagggagaagagggttagag

SEQ ID NO: 78 - DNA, 43 bp, synthetic construct
  source 1..43: mol_type = other DNA; note = primer
ctaaccaaattacctgtatacatcagctgtctgttgtgtcgtc

SEQ ID NO: 79 - DNA, 40 bp, synthetic construct
  source 1..40: mol_type = other DNA; note = primer
cttgtaggaagactcctgcagcaggaggtaagatgctggt

SEQ ID NO: 80 - DNA, 41 bp, synthetic construct
  source 1..41: mol_type = other DNA; note = primer
tgcaggagtcttcctacaagaggatatgtcctgttgaaagc

SEQ ID NO: 81 - DNA, 19 bp, synthetic construct
  source 1..19: mol_type = other DNA; note = primer
tgctcggccttgttctccc

SEQ ID NO: 82 - DNA, 22 bp, synthetic construct
  source 1..22: mol_type = other DNA; note = primer
aaatgccagcatgcagaatagg

SEQ ID NO: 83 - DNA, 19 bp, synthetic construct
  source 1..19: mol_type = other DNA; note = primer
tgctcggccttgttctccc

SEQ ID NO: 84 - DNA, 27 bp, synthetic construct
  source 1..27: mol_type = other DNA; note = primer
aaaaataccagcatgcagaataggtgc

SEQ ID NO: 85 - DNA, 22 bp, synthetic construct
  source 1..22: mol_type = other DNA; note = primer
cctattctgcatgctggcattt

SEQ ID NO: 86 - DNA, 20 bp, synthetic construct
  source 1..20: mol_type = other DNA; note = primer
gcatgtggcttcaaggcttg

SEQ ID NO: 87 - DNA, 22 bp, synthetic construct
  source 1..22: mol_type = other DNA; note = primer
cctattctgcatgctggtattt

SEQ ID NO: 88 - DNA, 20 bp, synthetic construct
  source 1..20: mol_type = other DNA; note = primer
gcatgtggcttcaaggcttg

SEQ ID NO: 89 - DNA, 20 bp, synthetic construct
  source 1..20: mol_type = other DNA; note = primer
caagccttgaagccacatgc

SEQ ID NO: 90 - DNA, 21 bp, synthetic construct
  source 1..21: mol_type = other DNA; note = primer
tcttgttgcccaaggggagtg

SEQ ID NO: 91 - DNA, 20 bp, synthetic construct
  source 1..20: mol_type = other DNA; note = primer
actccccttgggcaacaaga

SEQ ID NO: 92 - DNA, 22 bp, synthetic construct
  source 1..22: mol_type = other DNA; note = primer
tcttgacctcgtgaactgctcg

SEQ ID NO: 93 - DNA, 21 bp, synthetic construct
  source 1..21: mol_type = other DNA; note = primer
agcagttcacgaggtcaagaa

SEQ ID NO: 94 - DNA, 22 bp, synthetic construct
  source 1..22: mol_type = other DNA; note = primer
gggtcagatccgaataccacag

SEQ ID NO: 95 - DNA, 25 bp, synthetic construct
  source 1..25: mol_type = other DNA; note = primer
gaactgtggtattcggatctgaccc

SEQ ID NO: 96 - DNA, 19 bp, synthetic construct
  source 1..19: mol_type = other DNA; note = primer
cgtatgcagcccgagggtg

SEQ ID NO: 97 - DNA, 45 bp, synthetic construct
  source 1..45: mol_type = other DNA; note = primer
atgtacccatacgatgttccagattacgctgccatggatgagtat

SEQ ID NO: 98 - DNA, 40 bp, synthetic construct
  source 1..40: mol_type = other DNA; note = primer
gtctgttgtgtcgtcatctctaccaaccatggcactaact

SEQ ID NO: 99 - DNA, 40 bp, synthetic construct
  source 1..40: mol_type = other DNA; note = primer
agttagtgccatggttggtagagatgacgacacaacagac

SEQ ID NO: 100 - DNA, 40 bp, synthetic construct
  source 1..40: mol_type = other DNA; note = primer
cagctgccacacagcggaacctcctgctgcaggactcttc

SEQ ID NO: 101 - DNA, 40 bp, synthetic construct
  source 1..40: mol_type = other DNA; note = primer
gaagagtcctgcagcaggaggttccgctgtgtggcagctg

SEQ ID NO: 102 - DNA, 35 bp, synthetic construct
  source 1..35: mol_type = other DNA; note = primer
gagcggccgcgtacgcgtcacatatggaaggatcc

SEQ ID NO: 103 - DNA, 45 bp, synthetic construct; identical to SEQ ID NO: 97
  source 1..45: mol_type = other DNA; note = primer

SEQ ID NO: 104 - DNA, 59 bp, synthetic construct
  source 1..59: mol_type = other DNA; note = primer
aacctgtatacatcagctgtctgttgtgtcgtcatctctaccaaccatggcactaactt

SEQ ID NO: 105 - DNA, 58 bp, synthetic construct
  source 1..58: mol_type = other DNA; note = primer
ggtagagatgacgacacaacagacagctgatgtatacaggttccgctgtgtggcagct

SEQ ID NO: 106 - DNA, 35 bp, synthetic construct; identical to SEQ ID NO: 102
  source 1..35: mol_type = other DNA; note = primer

SEQ ID NO: 107 - DNA, 45 bp, synthetic construct; identical to SEQ ID NO: 97
  source 1..45: mol_type = other DNA; note = primer

SEQ ID NO: 108 - DNA, 40 bp, synthetic construct
  source 1..40: mol_type = other DNA; note = primer
tgggttgtttccactttgggctgttattttcctccgcatc

SEQ ID NO: 109 - DNA, 40 bp, synthetic construct
  source 1..40: mol_type = other DNA; note = primer
gatgcggaggaaaataacagcccaaagtggaaacaaccca

SEQ ID NO: 110 - DNA, 40 bp, synthetic construct
  source 1..40: mol_type = other DNA; note = primer
accttctttttgtaatttgccagcatgcagaataggtgct

SEQ ID NO: 111 - DNA, 40 bp, synthetic construct
  source 1..40: mol_type = other DNA; note = primer
agcacctattctgcatgctggcaaattacaaaaagaaggt

SEQ ID NO: 112 - DNA, 35 bp, synthetic construct; identical to SEQ ID NO: 102
  source 1..35: mol_type = other DNA; note = primer

SEQ ID NO: 113 - DNA, 20 bp, synthetic construct
  source 1..20: mol_type = other DNA; note = primer
caccgcggttccgaaggaat

SEQ ID NO: 114 - DNA, 20 bp, synthetic construct
  source 1..20: mol_type = other DNA; note = primer
tcggggactcactgcatcgt

SEQ ID NO: 115 - DNA, 25 bp, synthetic construct
  source 1..25: mol_type = other DNA; note = primer
caggtcctgcctcctcttgtgaatg

SEQ ID NO: 116 - DNA, 24 bp, synthetic construct
  source 1..24: mol_type = other DNA; note = primer
gggtttcgaggagctggctcgttt

SEQ ID NO: 117 - DNA, 294 bp, synthetic construct
  source 1..294: mol_type = other DNA; note = probe
accgtaaccaaacgaactgtaccgacagtagtttgaaagccagcagttagcagtttcttcagacttcaacactgtccagcgctttccagagcagactcactgtttacaagaactcttggcctcccgaagttagcaacctcagattttgtttatttaaagaatttctgtgaaagaaaaggaccccagagcccattttccaaaatggccatggacgggtatctgtggatggtcattttgggtttcattattgctttcatcctggcgttttcagtcggtgccaacgatgttgccaat

SEQ ID NO: 118 - DNA, 427 bp, synthetic construct
  source 1..427: mol_type = other DNA; note = probe
cttcactgagtattcctttcattccttcagtcgcctcctggtttatatcgccacttctttctggcttcatgtccggcgtgctgttcatactaatcagaatgttcatccttactaaggtgagtgtggcggcttctctggtttctgggttgtactaagttttagaactgattctggttctactcagtagaagctagtaccagtaccagtggctcggcaggagacctgtactttcattgccaggactcacctggagtttgagtcacgggtgttcaggaagggtcagaagcctcagggaacggccaagactctcccgggccttgcacacaagggcgcttccagccaggctctataatttacttcgttagcccaagctcccagaaattgggcttagacctcaagaatgaggtgattatttcctggttgtcaa

SEQ ID NO: 119 - DNA, 24 bp, synthetic construct
  source 1..24: mol_type = other DNA; note = primer
cccgaagttagcaacctcagattt

SEQ ID NO: 120 - DNA, 21 bp, synthetic construct
  source 1..21: mol_type = other DNA; note = primer
tcccactggtgccaatggagg

SEQ ID NO: 121 - DNA, 24 bp, synthetic construct
  source 1..24: mol_type = other DNA; note = primer
cccgaagttagcaacctcagattt

SEQ ID NO: 122 - DNA, 21 bp, synthetic construct
  source 1..21: mol_type = other DNA; note = primer
aaatgtgaaacatccaaccag

SEQ ID NO: 123 - DNA, 18 bp, synthetic construct
  source 1..18: mol_type = other DNA; note = primer
gcggccgggaattggatc

SEQ ID NO: 124 - DNA, 20 bp, synthetic construct
  source 1..20: mol_type = other DNA; note = primer
tcagctgccacacagcggaa

SEQ ID NO: 125 - DNA, 19 bp, synthetic construct
  source 1..19: mol_type = other DNA; note = primer
cgggaattggatcctgctc

SEQ ID NO: 126 - DNA, 20 bp, synthetic construct
  source 1..20: mol_type = other DNA; note = primer
accttactgaggctttcgtc

SEQ ID NO: 127 - DNA, 18 bp, synthetic construct
  source 1..18: mol_type = other DNA; note = primer
cggccgggaattggatcc

SEQ ID NO: 128 - DNA, 20 bp, synthetic construct
  source 1..20: mol_type = other DNA; note = primer
aggccacgaagatgttccga

SEQ ID NO: 129 - DNA, 19 bp, synthetic construct
  source 1..19: mol_type = other DNA; note = primer
tggccatggacgggtatct

SEQ ID NO: 130 - DNA, 19 bp, synthetic construct
  source 1..19: mol_type = other DNA; note = primer
gtatgaacagcacgccgga

SEQ ID NO: 131 - DNA, 20 bp, synthetic construct
  source 1..20: mol_type = other DNA; note = primer
ccttactaaggaggaccctg

SEQ ID NO: 132 - DNA, 20 bp, synthetic construct
  source 1..20: mol_type = other DNA; note = primer
tggacacacgaatagccaca

SEQ ID NO: 133 - DNA, 21 bp, synthetic construct
  source 1..21: mol_type = other DNA; note = primer
ctcggcctaatgtggtaggat

SEQ ID NO: 134 - DNA, 22 bp, synthetic construct
  source 1..22: mol_type = other DNA; note = primer
gggaaagctgtgatgtctcctc

SEQ ID NO: 135 - DNA, 20 bp, synthetic construct
  source 1..20: mol_type = other DNA; note = primer
cacagctttcccagatcggg

SEQ ID NO: 136 - DNA, 20 bp, synthetic construct
  source 1..20: mol_type = other DNA; note = primer
tcagctgccacacagcggaa

SEQ ID NO: 137 - DNA, 22 bp, synthetic construct
  source 1..22: mol_type = other DNA; note = primer
aggattctcactggtcgcaatc

SEQ ID NO: 138 - DNA, 20 bp, synthetic construct
  source 1..20: mol_type = other DNA; note = primer
gcaggccagacatgaaacca

SEQ ID NO: 139 - DNA, 19 bp, synthetic construct
  source 1..19: mol_type = other DNA; note = primer
tttcatgtctggcctgctg

SEQ ID NO: 140 - DNA, 22 bp, synthetic construct
  source 1..22: mol_type = other DNA; note = primer
ggtagcagcatagaatactggg

SEQ ID NO: 141 - DNA, 20 bp, synthetic construct
  source 1..20: mol_type = other DNA; note = primer
tccgggcactcccagtattc

SEQ ID NO: 142 - DNA, 19 bp, synthetic construct
  source 1..19: mol_type = other DNA; note = primer
tgagggctatggcccacat

SEQ ID NO: 143 - DNA, 20 bp, synthetic construct
  source 1..20: mol_type = other DNA; note = primer
gccatagccctcatttcctt

SEQ ID NO: 144 - DNA, 21 bp, synthetic construct
  source 1..21: mol_type = other DNA; note = primer
actcgtgataaagcaccttct

SEQ ID NO: 145 - DNA, 21 bp, synthetic construct
  source 1..21: mol_type = other DNA; note = primer
ggtgccaaggctaatgatgac

SEQ ID NO: 146 - DNA, 20 bp, synthetic construct
  source 1..20: mol_type = other DNA; note = primer
tgggtcatggacagtgctct

SEQ ID NO: 147 - DNA, 21 bp, synthetic construct
  source 1..21: mol_type = other DNA; note = primer
ctgtttcgggtcctttgctca

SEQ ID NO: 148 - DNA, 20 bp, synthetic construct
  source 1..20: mol_type = other DNA; note = primer
ataaaacagcagccagacgg

SEQ ID NO: 149 - DNA, 19 bp, synthetic construct
  source 1..19: mol_type = other DNA; note = primer
tgatccagaccatggggaa

SEQ ID NO: 150 - DNA, 19 bp, synthetic construct
  source 1..19: mol_type = other DNA; note = primer
tgactggaagcccgatgtt

SEQ ID NO: 151 - DNA, 20 bp, synthetic construct
  source 1..20: mol_type = other DNA; note = primer
tcagcaccacgcactgtaag

SEQ ID NO: 152 - DNA, 19 bp, synthetic construct
  source 1..19: mol_type = other DNA; note = primer
ccacagggacggtcacgaa

SEQ ID NO: 153 - protein, 696 aa, synthetic construct
  source 1..696: note; note (original language) = 人XPR1蛋白序列
MKFAEHLSAHITPEWRKQYIQYEAFKDMLYSAQDQAPSVEVTDEDTVKRYFAKFEEKFFQTCEKELAKINTFYSEKLAEAQRRFATLQNELQSSLDAQKESTGVTTLRQRRKPVFHLSHEERVQHRNIKDLKLAFSEFYLSLILLQNYQNLNFTGFRKILKKHDKILETSRGADWRVAHVEVAPFYTCKKINQLISETEAVVTNELEDGDRQKAMKRLRVPPLGAAQPAPAWTTFRVGLFCGIFIVLNITLVLAAVFKLETDRSIWPLIRIYRGGFLLIEFLFLLGINTYGWRQAGVNHVLIFELNPRSNLSHQHLFEIAGFLGILWCLSLLACFFAPISVIPTYVYPLALYGFMVFFLINPTKTFYYKSRFWLLKLLFRVFTAPFHKVGFADFWLADQLNSLSVILMDLEYMICFYSLELKWDESKGLLPNNSEESGICHKYTYGVRAIVQCIPAWLRFIQCLRRYRDTKRAFPHLVNAGKYSTTFFMVTFAALYSTHKERGHSDTMVFFYLWIVFYIISSCYTLIWDLKMDWGLFDKNAGENTFLREEIVYPQKAYYYCAIIEDVILRFAWTIQISITSTTLLPHSGDIIATVFAPLEVFRRFVWNFFRLENEHLNNCGEFRAVRDISVAPLNADDQTLLEQMMDQDDGVRNRQKNRSWKYNQSISLRRPRLASQSKARDTKVLIEDTDDEANT

SEQ ID NO: 154 - protein, 714 aa, synthetic construct
  source 1..714: note; note (original language) = 人MYORG蛋白序列
MLQNPQEKSQAYPRRRRPGCYAYRQNPEAIAAAAMYTFLPDNFSPAKPKPSKDLKPLLGSAVLGLLLVLAAVVAWCYYSVSLRKAERLRAELLDLKAGGFSIRNQKGEQVFRLAFRSGALDLDSCSRDGALLGCSLTADGLPLHFFIQTVRPKDTVMCYRVRWEEAAPGRAVEHAMFLGDAAAHWYGGAEMRTQHWPIRLDGQQEPQPFVTSDVYSSDAAFGGILERYWLSSRAAAIKVNDSVPFHLGWNSTERSLRLQARYHDTPYKPPAGRAAAPELSYRVCVGSDVTSIHKYMVRRYFNKPSRVPAPEAFRDPIWSTWALYGRAVDQDKVLRFAQQIRLHHFNSSHLEIDDMYTPAYGDFDFDEVKFPNASDMFRRLRDAGFRVTLWVHPFVNYNSSRFGEGVERELFVREPTGRLPALVRWWNGIGAVLDFTHPKARDWFQGHLRRLRSRYSVASFKFDAGEVSYLPRDFSTYRPLPDPSVWSRRYTEMALPFFSLAEVRVGYQSQNISCFFRLVDRDSVWGYDLGLRSLIPAVLTVSMLGYPFILPDMVGGNAVPQRTAGGDVPERELYIRWLEVAAFMPAMQFSIPPWRYDAEVVAIAQKFAALRASLVAPLLLELAGEVTDTGDPIVRPLWWIAPGDETAHRIDSQFLIGDTLLVAPVLEPGKQERDVYLPAGKWRSYKGELFDKTPVLLTDYPVDLDEIAYFTWAS

SEQ ID NO: 155 - protein, 652 aa, synthetic construct
  source 1..652: note; note (original language) = 人PiT2蛋白序列
MAMDEYLWMVILGFIIAFILAFSVGANDVANSFGTAVGSGVVTLRQACILASIFETTGSVLLGAKVGETIRKGIIDVNLYNETVETLMAGEVSAMVGSAVWQLIASFLRLPISGTHCIVGSTIGFSLVAIGTKGVQWMELVKIVASWFISPLLSGFMSGLLFVLIRIFILKKEDPVPNGLRALPVFYAATIAINVFSIMYTGAPVLGLVLPMWAIALISFGVALLFAFFVWLFVCPWMRRKITGKLQKEGALSRVSDESLSKVQEAESPVFKELPGAKANDDSTIPLTGAAGETLGTSEGTSAGSHPRAAYGRALSMTHGSVKSPISNGTFGFDGHTRSDGHVYHTVHKDSGLYKDLLHKIHIDRGPEEKPAQESNYRLLRRNNSYTCYTAAICGLPVHATFRAADSSAPEDSEKLVGDTVSYSKKRLRYDSYSSYCNAVAEAEIEAEEGGVEMKLASELADPDQPREDPAEEEKEEKDAPEVHLLFHFLQVLTACFGSFAHGGNDVSNAIGPLVALWLIYKQGGVTQEAATPVWLLFYGGVGICTGLWVWGRRVIQTMGKDLTPITPSSGFTIELASAFTVVIASNIGLPVSTTHCKVGSVVAVGWIRSRKAVDWRLFRNIFVAWFVTVPVAGLFSAAVMALLMYGILPYV

SEQ ID NO: 156 - DNA, 992 bp, synthetic construct
  source 1..992: mol_type = other DNA; note; note (original language) = gfaABC1D启动子序列
taacatatcctggtgtggagtaggggacgctgctctgacagaggctcgggggcctgagctggctctgtgagctggggaggaggcagacagccaggccttgtctgcaagcagacctggcagcattgggctggccgccccccagggcctcctcttcatgcccagtgaatgactcaccttggcacagacacaatgttcggggtgggcacagtgcctgcttcccgccgcaccccagcccccctcaaatgccttccgagaagcccattgagcagggggcttgcattgcaccccagcctgacagcctggcatcttgggataaaagcagcacagccccctaggggctgcccttgctgtgtggcgccaccggcggtggagaacaaggctctattcagcctgtgcccaggaaaggggatcaggggatgcccaggcatggacagtgggtggcagggggggagaggagggctgtctgcttcccagaagtccaaggacacaaatgggtgaggggagagctctccccatagctgggctgcggcccaaccccaccccctcaggctatgccagggggtgttgccaggggcacccgggcatcgccagtctagcccactccttcataaagccctcgcatcccaggagcgagcagagccagagcaggttggagaggagacgcatcacctccgctgctcgcaagctttattgcggtagtttatcacagttaaattgctaacgcagtcagtgcttctgacacaacagtctcgaacttaagctgcagaagttggtcgtgaggcactgggcaggtaagtatcaaggttacaagacaggtttaaggagaccaatagaaactgggcttgtcgagacagagaagactcttgcgtttctgataggcacctattggtcttactgacatccactttgcctttctctccacaggtgtccactcccagttcaattacagctcttaaggctagagtacttaatacgactcactataggctagc